European Patent Application EP 4 151 732 A1, published March 22, 2023. Title: TRANSGENIC PLANTS PRODUCING HIGH LEVELS OF APOCAROTENOIDS COMPOUNDS AND USES THEREOF. Applicant: Consejo Superior de Investigaciones Científicas (CSIC) Universidad Castilla La Mancha (UCLM). The sequence listing filed with the application follows.

SEQUENCE LISTING (32 sequences)

SEQ ID NO: 1 - DNA, 1898 bp, Crocus sativus
  CDS (16)..(1887)
actattattcttgacatggaatctcctgctactaaattacctgcacctctgctgatgttatcttcttctccattccttctcccttctcctaataagagctcctccatcttccttccacgtaaattagggccgctacctccaaaatattattattacaattgctgccatcctaagagtagatcaatctcagtagtatcaatggcaaataaggaggaggcagagaccagtaagaagaagcccaaaccattaaaagtactaattaccaaagtggatccgaagccgaggaagggcatggcatccgtcgcagtggacttactcgagaaggcctttgtatacctattgtccggaaattctgcagctgatcgtagtagtagtagtggtcgtcgtcgtcgtaaagagcattactacctctccggcaattatgcgcccgtcggacacgaaaccccgccctccgaccacctccccattcatggatcccttcctgaatgcttgaatggagtgtttctgagagttggtcctaaccccaagtttgctcccgtagccggatacaattgggtcgatggagatggaatgattcatggattgcgtattaaagatggaaaagcaacttatctatctcgatatattaaaacgtcacggtttaaacaagaagaatattttggaagagcaaaatttatgaagattggagatctaaggggattgcttgggttctttacgatcttaatactagtacttcgaacaacattgaaagtaatagacatttcatatggaagagggacgggtaatacagctcttgtgtatcataatggcttactattggctctatcagaagaagataaaccttatgttgttaaagttttagaagatggagacttgcaaactcttgggatattggattatgacaagaaattgtcacatccattcaccgctcatccaaagatcgatccgttaactgatgagatgtttacctttggatattccatctcgcctccgtatcttacttatcgagtcatttccaaggatggagtgatgcaagatccagtgcaaatctcaattacatcccctaccataatgcatgattttgctattactgaaaattatgccatcttcatggacctgcccttgtatttccaaccagaggaaatggtaaaggggaaatttgtctcttcatttcaccctacaaaaagagctcgtatcggtgtgcttccacgatatgcaaaagacgagcatccaattcgatggttcgatcttccaagttgcttcatgactcataatgcaaatgcttgggaagagaatgatgaagttgtgctattcacatgtcgccttgagagtcctgatcttgacatgcttagtggacctgcggaagaagagattgggaattcaaaaagtgagctttacgaaatgaggttcaatttgaaaactggaattacttcacaaaagcaactatctgtacctagtgttgattttcctcggatcaaccaaagttatactggcaggaaacagcaatatgtttattgtactcttggcaacaccaagattaagggcattgtgaagtttgatctgcaaattgaaccagaagccggaaagacaatgcttgaagttggaggaaatgtacaaggcatctttgagttgggacctagaagatatggttcagaggcaatatttgtgccatgccaacctggcatcaaatctgatgaggatgacggttacttgatattctttgtacacgacgaaaacaatgggaaatctgaggtcaatgtcatcgatgcaaagacaatgtctgcagaacctgtggctgttgtggaacttccaagcagggttccatatggattccatgccttgtttctgaatgaggaagaacttcagaagcaccaagcagagacatgacaatcactagt

SEQ ID NO: 2 - protein, 623 aa, Crocus sativus
MESPATKLPAPLLMLSSSPFLLPSPNKSSSIFLPRKLGPLPPKYYYYNCCHPKSRSISVVSMANKEEAETSKKKPKPLKVLITKVDPKPRKGMASVAVDLLEKAFVYLLSGNSAADRSSSSGRRRRKEHYYLSGNYAPVGHETPPSDHLPIHGSLPECLNGVFLRVGPNPKFAPVAGYNWVDGDGMIHGLRIKDGKATYLSRYIKTSRFKQEEYFGRAKFMKIGDLRGLLGFFTILILVLRTTLKVIDISYGRGTGNTALVYHNGLLLALSEEDKPYVVKVLEDGDLQTLGILDYDKKLSHPFTAHPKIDPLTDEMFTFGYSISPPYLTYRVISKDGVMQDPVQISITSPTIMHDFAITENYAIFMDLPLYFQPEEMVKGKFVSSFHPTKRARIGVLPRYAKDEHPIRWFDLPSCFMTHNANAWEENDEVVLFTCRLESPDLDMLSGPAEEEIGNSKSELYEMRFNLKTGITSQKQLSVPSVDFPRINQSYTGRKQQYVYCTLGNTKIKGIVKFDLQIEPEAGKTMLEVGGNVQGIFELGPRRYGSEAIFVPCQPGIKSDEDDGYLIFFVHDENNGKSEVNVIDAKTMSAEPVAVVELPSRVPYGFHALFLNEEELQKHQAET

SEQ ID NO: 3 - DNA, 1496 bp, Crocus sativus
  CDS (35)..(1417)
ggacagccagcagaaatcacaatggacgagaaagatgttgaacggcaacaaatgccacatcctcctcctcccctgtccagcacaaggccatatcaaccccattctccaattcggcaagcgactggcctctcacaacctcctcaccacactcgtcaacacccggttcctctccaactcgaccaaatccgaacccggtccggtcaacatccagtgcatatccgacggattcgatcccggtgggatgaatgcagcacctagtcgtcgggcctatttcgaccgacctcagagtcggtcgggtcagaaacatgttggcctcatcgagtcactccggtccagaggccgacccggcgcatgttttggtctacgacccgttcccctctgggcaatgaacgtagccgagcggtccgggctgcggtcggtcgcattctttactcagccgtgtgcagtggacacaatctaccgccacgtgtgggagggacgaattaaggttccggttgccgagccggtccggttgcctggattgcccccactcgagcctagtgatctgccgtgcgttcgtaacggattcggacgagtcgttaacccggatctcttgccacttcgagtgaatcagcacaaaaatttggacaaagctgacatgatggggaggaactccatatacgagctagaggcggatttgttggatgggtcccgattaccattaccggtgaagtcgattgggccgaccgtgccgtctacttatctcgacaaccgaatcccgtcggattcacactatggattcaatctatacacccctgacactactccctacttggactggctcgactccaaggccccgaactctgtcatctatgtctcatttggtagtttgtccagtctgagccctgatcaaaccaatgagattgcgtcgggtctgatcgccaccaacaaaagctttatttgggtggtacgcacttcggagttagccaaactccctgccaacttcacccaagagaatgcgagccgtgggctggttgtgacctggtgcgaccaactcgatctcctcgcacacgttgcgaccggttgcttcgtgactcactgcggatggaactcgactatggaaggtgtcgcacttggtgtgccgatggtgggagtgccgcagtggtcggaccagcctatgaatgccaagtatgtagaggatgtgtggaaggtcggcgtgagggcgaagacttatgggaaggattttgtgagaggggaggagttcaaaagatgtgtggaggaggtgatggatggagagaggagtggaaagattagagagaatgccgcaaggtggtgtaagttggccaaggactctgttagtgagggtgggagttctgacaagtgtatcaaggagttcatacatcagtgttgcaatgactccaaaatttccttagtttaatcaccctgttaataaagttttgtttcatgtgtcaaacctgagtcaatctattaagagaaaaattgtgcataacagaaga

SEQ ID NO: 4 - protein, 460 aa, Crocus sativus
MLNGNKCHILLLPCPAQGHINPILQFGKRLASHNLLTTLVNTRFLSNSTKSEPGPVNIQCISDGFDPGGMNAAPSRRAYFDRPQSRSGQKHVGLIESLRSRGRPGACFGLRPVPLWAMNVAERSGLRSVAFFTQPCAVDTIYRHVWEGRIKVPVAEPVRLPGLPPLEPSDLPCVRNGFGRVVNPDLLPLRVNQHKNLDKADMMGRNSIYELEADLLDGSRLPLPVKSIGPTVPSTYLDNRIPSDSHYGFNLYTPDTTPYLDWLDSKAPNSVIYVSFGSLSSLSPDQTNEIASGLIATNKSFIWVVRTSELAKLPANFTQENASRGLVVTWCDQLDLLAHVATGCFVTHCGWNSTMEGVALGVPMVGVPQWSDQPMNAKYVEDVWKVGVRAKTYGKDFVRGEEFKRCVEEVMDGERSGKIRENAARWCKLAKDSVSEGGSSDKCIKEFIHQCCNDSKISLV

SEQ ID NO: 5 - DNA, 1548 bp, Crocus sativus
  CDS (1)..(1548)
atggctgagaaagaagcaaatacccatgtcgtcctcttccccttgccaggccaagggcacatcggctcaatgctgaaactggcacagcttctttccaccgccggattctacgtcactttcgtccacaccgaacgcaactaccgtcgctacctcctcacctccacgtccttccacgtccccaagttccggttccgcaccatccccgacggttttcccgacgacgattcccgctcgcccctcccttttctcgagctccaagagtcgctggacacgaaatgtcgggggcattatcgggaattgttggtcgctgtcgacgaccaagaagagtggcccccagtcacttgtgtcgtggctgatcaagctcttccactctcactcgaagttcccgacgagttggggattcctgtaatgatactcgcaccacacagtgcgtgcagtatattgacgagttattcgattccggagcttataaggggaggtgaactccctatcccagatggggccaatatggatgaactattacaaggcgtactgggattggaaggtatcgtgaggcgtagggatatgtccatcagaagcgccaagtccatccaagatccatttcttcaattcgaagtgaaaatgagcaaaaacttgcccagaggaagagctctcatcctgaacactacagaatcgatagactctctttctttgcgacacattcggtcgatctgtcccactacctacgcactcgggcccttccacgtccttctcaggaacataaaagacgagtcccactccgcaagcctttccgaagaggacaggtcctgcatcgcctggctggactcgaaaccgaacaagtccgcggtctacgtgagtttcggtagcctcgccgccatgccgagagaagcatttcttgagtttcagcagggattgctcgacagcgggtattacttcttgtgggtgatccggcccgatatggtggaaggggggctggaagagagcgagctgaccgcgagcgaacaacgctactttgtgaagtgggccccacaggaggaggttcttgcgcacccggcggtagggtgtttcttgacgcacagcggttggaactctacgttggagagtatctttgcgggagtgccgatgatatgttggcctttctttgcggaccagctgattaacagtaggtttgcgagcgaggtgtggaaaattgccttggatatgaaggatttatgcggaaggagccacgtggagaggatggtgaaggaagttatgagtggagagaaaggcgaagagctaaggaattctagctgcgagatggcagatagggtgaagaagagtgcagaggaaggtggctcttcctatgccaacttcaaagagttggttggacatatcaaatctttgagcttaccagcagaaagaggagaaaatggtggtgaaggaatgagtgtacaagcgccgagtaaacttttcctcctcaacgctgaggacggaaaacatgtccttaaaagtgacgaaccgtcggaacaaaggggtccacaatttaatccaaattttcttcggacctga

SEQ ID NO: 6 - protein, 515 aa, Crocus sativus
MAEKEANTHVVLFPLPGQGHIGSMLKLAQLLSTAGFYVTFVHTERNYRRYLLTSTSFHVPKFRFRTIPDGFPDDDSRSPLPFLELQESLDTKCRGHYRELLVAVDDQEEWPPVTCVVADQALPLSLEVPDELGIPVMILAPHSACSILTSYSIPELIRGGELPIPDGANMDELLQGVLGLEGIVRRRDMSIRSAKSIQDPFLQFEVKMSKNLPRGRALILNTTESIDSLSLRHIRSICPTTYALGPFHVLLRNIKDESHSASLSEEDRSCIAWLDSKPNKSAVYVSFGSLAAMPREAFLEFQQGLLDSGYYFLWVIRPDMVEGGLEESELTASEQRYFVKWAPQEEVLAHPAVGCFLTHSGWNSTLESIFAGVPMICWPFFADQLINSRFASEVWKIALDMKDLCGRSHVERMVKEVMSGEKGEELRNSSCEMADRVKKSAEEGGSSYANFKELVGHIKSLSLPAERGENGGEGMSVQAPSKLFLLNAEDGKHVLKSDEPSEQRGPQFNPNFLRT

SEQ ID NO: 7 - DNA, 2157 bp, Artificial Sequence
  pE8 promoter
tccctaatgatattgttcacgtaattaagttttgtggaagtgagagagtccaattttgataagaaaagagtcagaaaacgtaatattttaaaagtctaaatctttctacaaataagagcaaatttatttattttttaatccaataaatattaatggaggacaaattcaattcacttggttgtaaaataaacttaaaccaataaccaaagaactaataaatcctgaagtggaattattaaggataaatgtacatagacaatgaagaaataataggttcgatgaattaataataattaaggatgttacaatcatcatgtgccaagtatatacacaatattctatgggatttataatttcgttacttcacttaacttttgcgtaaataaaacgaattatctgatattttataataaaacagttataagaaccatcatttttaacaacatagatatattatttctaatagtttaatgatacttttaaatcttttaaattttatgtttcttttagaaaataaaaattcaaaaaattaaatatatttacaaaaactacaatcaaacacaacttcatatattaaaagcaaaatatattttgaaaatttcaagtgtcctaacaaataagacaagaggaaaatgtacgatgagagacataaagagaactaataattgaggagtcctataatatataataaagtttattagtaaacttaattattaaggactcctaaaatatatgataggagaaaatgaatggtgagagatattggaaaacttaataattaaggattttaaaatatatggtaaaagataggcaaagtatccattatccccttttaacttgaagtctactaggcgcatgtgaaagttgattttttgtcacgtcatatagctataacgtaaaaaaagaaagtaaaatttttaattttttttaatatatgacatattttaaacgaaatataggacaaaatgtaaatgaatagtaaaggaaacaaagattaatacttactttgtaagaatttaagataaatttaaaatttaatagatcaactttacgtctagaaagacccatatctagaaggaatttcacgaaatcggcccttattcgaaaataacttttaaataatgaattttaaattttaagaaataatatccaatgaataaatgacatgtagcattttacctaaatatttcaactattttaatccaatattaatttgttttattcccaacaatagaaagtcttgtgcagacatttaatctgacttttccagtactaaatattaattttctgaagattttcgggtttagtccacaagttttagtgagaagttttgctcaaattttaggtgagaaggtttgatatttatcttttgttaaattaatttatctaggtgactattatttatttaagtagaaattcatatcattacttttgccaacttgtagtcataataggagtaggtgtatatgatgaaggaataaacaagttcagtgaagtgattaaaataaaatataatttaggtgtacatcaaataaaaaccttaaagtttagaaaggcaccgaataattttgcatagaagatattagtaaatttataaaaataaaagaaatgtagttgtcaagttgtcttcttttttttggataaaaatagcagttggcttatgtcattcttttacaacctccatgccacttgtccaattgttgacacttaactaattagtttgattcatgtatgaatactaaataattttttaggactgactcaaatatttttatattatcatagtaatatttatctaatttttaggaccacttattactaaataataaattaactacaactatattattgttgtgaaacaacaacgttttggttgttatgatgaaacgtacactatatcagtatgaaaaattcaaaacgattagtataaattatattgaaaatttgatatttttctattcttaatcagacgtattgggtttcatattttaaaaagggactaaacttagaagagaagtttgtttgaaactacttttgtctctttcttgttcccatttctctcttagatttcaaaaagtgaactactttatctccttctttgttcacattttattttattctattataaatatggcatcctcatattgagatttttag

SEQ ID NO: 8 - DNA, 4034 bp, Artificial Sequence
  p2A11 promoter
gtcaaacaattttgaggaattcaatttcatctttaactggtacaataatcattttatcatgaaaataagcagctcaagagaatttttgaagaatcttttatttctttaacatttaaccacatgaatttttaatttttttttgcaatacatttaaaccgaaatggtcaaacgatcaaccaactgatctttattctaataaacttctagtttacatttgcatgtgagtgcatcatcattatcatatttgtacacaacaaacaagaaaaaaatataaacaatattttatttaaatatttatattccactttgactgtagatattaaatcttgtcatcatttatagtctcaatattataatttttttattttttcaaaattcaaaagtttacaattatttttttgaactataatattatccaagatgaacatctcaagaagaaaattattaatattgttatggttaaaattttacatacaatacttgttttttgctttacttttatcttaccgtagatacacaatcgacgataacttagtgatcacacaataataattattttgttcatgacacaatatttataagaaatacttatttctttcttttatccttcagtagttcataataaaaacataccataatatttgtgatgcattcatagtacgtaatgaaatgacaatttatgtcaaattattttcttttatactctcaaacctcccgtaaaggtgagatgagtcatttatccaattatacataaatatgtctttattcatgctctttatcacattctgacacattcacttaatttcaagagtaagcaagcatgataactgaaactatttatgcgtatcttaccttgatatttgacacattacatgacacacctcaacatcactttcaaagattaagcgcaccaccatattatctttctttttttttttatgaaggttttataaaattattaaattaggtccaaaaaattgtttgtcaaataaccttttatactagattgatgacaaaaattacctttacgttttgaaagaccattttaagacctaatctatcagtgactccttaaagttggcacaatatttcacttagacaccctaattgaatgatgttcattttaaacacccaatgtagggttccgctatatcattttgacacatttcttaacatcaacaaaaatatataatgagtatgtgatatactcgcgaatgacgtgaaaaatgaagacatttgttatttgtatcaaagtagttactaaataattaattttgaataaaaataaaagctgaccagtaaatcaataacacataatattttccacctaataattaaaatataaaataaaaaagagccatctcagggtcatctgcccaccattgctatttcaaagaaatttgtacgttagtttatagaaattgatgttaaaattctttcaagaaaaatttatgaatgaatttattctctaatttaaaaatattttctgttatttttgttgaaagaaatttaacttggataaaatggtggttaaaactggaaagaagaaaagagaaaaaataattaaaaatcatttcacgctctaatcaatgagcgtatcacattcattatgttatataagcaaaagtgacaaaacgaaaataatatattacatgaaatgtctaaaataaatatcgtctaattaaaatatctaagtaacatattgtgcctaactttagagggatcatcaataagttaaaccccattttaataactcataattgtcctttttatttaatattgtcacaaatcacaatgataattaacattaatttgtcctttgtgacgtccatattcatgcatttaaccaatcatcttcatttggacttattatcacaattatcccactttcctcacaaaatggagcattcaagtggaatagactacacgatttttaatttcatcaaaaacatctttttgctttattcattattatattgtcgctattgttgaattttatttgccctaaatttcttaccataaatagatttttcttttagaaaaaggagattgactaattcttttcttgtaggaaaaggtttaggactctataaatagagacatattccttctaacttaatcaacatttacaatgtagtcttaaagactttgaaagtttttggttagggggagaaattgtgggtcacaagcttgatacgttatcaattgtgtaaacctcccatgtattctgagtgaatttggttgaggttgtttccctctgtattttgtactctcatatttatagtggattgttcatctctttcgtggacgtaggtcgattgaccgtcgattgaccgaaccacgttaaatctttgtattttttgatatatttctcattatcttcttactcgtgatctttcaaggtttgcattgctatcttccgcgttacaccaacttatttacgatcctaacagctatggtgtggaaacataaatcaaacattttactgatataaacacatctttgattataacatgatagaaatttgagcccaactttttatcatcattatatacaaaaagttctaaattttttttttgatgtagtaaaacttaaatccatagtcttgcccctaaaccaatgacataatatataacccaaaatatactagttttcgccctcgagccctttaaaaagtatagtcaatatttacggtgaccgtgaatttcttaattatgatatataatttaaaagaaatcatgatcacattctactgatgagaacatgtgctaatcaagggaaaacatggatgtgaaaaatactttttgttaaaagtaaaaaaaaatgtgaaattttgttagttatttactacctatacattatttgagcatgtgcaaactttacaaatacctaatagaagattttcacctgcctgtatatatgtaaattaattataatgaacactctcacataaaataattatcagtatatacattaatacttgccctccacaatgaattaaataaaatgtagaacatgatctacacttcaataaaactaagaccataaagaataatttcaaaatatacacatgtcaacaataaattatttgcatattatattaacttactaaacaatctttacttttgaaatataaaaataatcaagttataagtctgctcaaagtaaagcacttgttagactcatctgattttgagaaggtaagcaaattgatggtgcataatagtcacaagtaaaatataaaatagatttcattagtaaaattgttttttactttctttatatataattatcaatatccttcaatggtaggttaattatattgttaacttcttgttgaattaaagcaataagacaagaatattaaagataaaagaacaataaaaatagaaagactaagagataagagttttcttattcttctttcaataagtatcatcaagtgtatacaatataaatttttgtatttttgatctatctatttataatgttatatataagcatacaaaagatcagtcataaatatgactttaatcatgaaaataatgaaagagattatgaaggcgtaaggttactagaataatagtcattaaaaaaaggggttatctttataattgaataattgatgaagtaatggagataattagtgagcataaatttttttaaaaaaatggacatttacactataatattttataacactttcccttaaacatctaggtataaataatgagtcttgtcaaaatcttagtaggaaaaattctgtgaaatttttttagtgaaaacaaatgatataaatatcttgaatactcattatttgttgtctcattaaaaatcttatctgacctataaaataaattatttgctcaactcaaaatagtttttcattctaaaattagtataattattagtgaatatttaattaacataattgtatactaaggggcctataaattggattcttctcaaagaaaaataaaatcaccacacaactttcttcttctgctcatcaattagcaattaatccaaaacca

SEQ ID NO: 9 - DNA, 1027 bp, Artificial Sequence
  p35S promoter
actagagccaagctgatctcctttgccccggagatcaccatggacgactttctctatctctacgatctaggaagaaagttcgacggagaaggtgacgataccatgttcaccaccgataatgagaagattagcctcttcaatttcagaaagaatgctgacccacagatggttagagaggcctacgcggcaggtctgatcaagacgatctacccgagtaataatctccaggagatcaaataccttcccaagaaggttaaagatgcagtcaaaagattcaggactaactgcatcaagaacacagagaaagatatatttctcaagatcagaagtactattccagtatggacgattcaaggcttgcttcataaaccaaggcaagtaatagagattggagtctctaagaaagtagttcctactgaatcaaaggccatggagtcaaaaattcagatcgaggatctaacagaactcgccgtgaagactggcgaacagttcatacagagtcttttacgactcaatgacaagaagaaaatcttcgtcaacatggtggagcacgacactctcgtctactccaagaatatcaaagatacagtctcagaagaccaaagggctattgagacttttcaacaaagggtaatatcgggaaacctcctcggattccattgcccagctatctgtcacttcatcaaaaggacagtagaaaaggaaggtggcacctacaaatgccatcattgcgataaaggaaaggctatcgttcaagatgcctctgccgacagtggtcccaaagatggacccccacccacgaggagcatcgtggaaaaagaagacgttccaaccacgtcttcaaagcaagtggattgatgtgatatctccactgacgtaagggatgacgcacaatcccactatccttcgcaagacccttcctctatataaggaagttcatttcatttggagaggactccggtatttttacaacaataccacaacaaaacaaacaacaaacaacattacaatttactattctagtcga

SEQ ID NO: 10 - DNA, 37 bp, Artificial Sequence
  Primer pUPD2-Dom-UGT2-F
gcgccgtctcgctcgaatgttgaacggcaacaaatgc

SEQ ID NO: 11 - DNA, 45 bp, Artificial Sequence
  Primer pUPD2-Dom-UGT2-R
gcgccgtctcgctcaaagcttaaactaaggaaattttggagtcat

SEQ ID NO: 12 - DNA, 40 bp, Artificial Sequence
  Primer pUPD2-Dom-CsCCD2-L-F1
gcgccgtctcgctcgaatggaatctcctgctactaaatta

SEQ ID NO: 13 - DNA, 31 bp, Artificial Sequence
  Primer pUPD2-Dom-CsCCD2-L-R1
gcgccgtctcgttgtctctgcctcctcctta

SEQ ID NO: 14 - DNA, 33 bp, Artificial Sequence
  Primer pUPD2-Dom-CsCCD2-L-F2
gcgccgtctcgacaagtaagaagaagcccaaac

SEQ ID NO: 15 - DNA, 39 bp, Artificial Sequence
  Primer pUPD2-Dom-CsCCD2-L-R2
gcgccgtctcgctcaaagctcatgtctctgcttggtgct

SEQ ID NO: 16 - DNA, 39 bp, Artificial Sequence
  Primer pUPD2-Dom-UGT709-F
gcgccgtctcgctcgaatggctgagaaagaagcaaatac

SEQ ID NO: 17 - DNA, 40 bp, Artificial Sequence
  Primer pUPD2-Dom-UGT709-R
gcgccgtctcgctcaaagctcaggtccgaagaaaatttgg

SEQ ID NO: 18 - DNA, 3978 bp, Artificial Sequence
  Plasmid pUPD2-CsCCD2L
aatggaatctcctgctactaaattacctgcacctctgctgatgttatcttcttctccattccttctcccttctcctaataagagctcctccatcttccttccacgtaaattagggccgctacctccaaaatattattattacaattgctgccatcctaagagtagatcaatctcagtagtatcaatggcaaataaggaggaggcagagacaagtaagaagaagcccaaaccattaaaagtactaattaccaaagtggatccgaagccgaggaagggcatggcatccgtcgcagtggacttactcgagaaggcctttgtatacctattgtccggaaattctgcagctgatcgtagtagtagtagtggtcgtcgtcgtcgtaaagagcattactacctctccggcaattatgcgcccgtcggacacgaaaccccgccctccgaccacctccccattcatggatcccttcctgaatgcttgaatggagtgtttctgagagttggtcctaaccccaagtttgctcccgtagccggatacaattgggtcgatggagatggaatgattcatggattgcgtattaaagatggaaaagcaacttatctatctcgatatattaaaacgtcacggtttaaacaagaagaatattttggaagagcaaaatttatgaagattggagatctaaggggattgcttgggttctttacgatcttaatactagtacttcgaacaacattgaaagtaatagacatttcatatggaagagggacgggtaatacagctcttgtgtatcataatggcttactattggctctatcagaagaagataaaccttatgttgttaaagttttagaagatggagacttgcaaactcttgggatattggattatgacaagaaattgtcacatccattcaccgctcatccaaagatcgatccgttaactgatgagatgtttacctttggatattccatctcgcctccgtatcttacttatcgagtcatttccaaggatggagtgatgcaagatccagtgcaaatctcaattacatcccctaccataatgcatgattttgctattactgaaaattatgccatcttcatggacctgcccttgtatttccaaccagaggaaatggtaaaggggaaatttgtctcttcatttcaccctacaaaaagagctcgtatcggtgtgcttccacgatatgcaaaagacgagcatccaattcgatggttcgatcttccaagttgcttcatgactcataatgcaaatgcttgggaagagaatgatgaagttgtgctattcacatgtcgccttgagagtcctgatcttgacatgcttagtggacctgcggaagaagagattgggaattcaaaaagtgagctttacgaaatgaggttcaatttgaaaactggaattacttcacaaaagcaactatctgtacctagtgttgattttcctcggatcaaccaaagttatactggcaggaaacagcaatatgtttattgtactcttggcaacaccaagattaagggcattgtgaagtttgatctgcaaattgaaccagaagccggaaagacaatgcttgaagttggaggaaatgtacaaggcatctttgagttgggacctagaagatatggttcagaggcaatatttgtgccatgccaacctggcatcaaatctgatgaggatgacggttacttgatattctttgtacacgacgaaaacaatgggaaatctgaggtcaatgtcatcgatgcaaagacaatgtctgcagaacctgtggctgttgtggaacttccaagcagggttccatatggattccatgccttgtttctgaatgaggaagaacttcagaagcaccaagcagagacatgagctttgagaccactcatcgcgactagtagcggccgctgcagtccggcaaaaaagggcaaggtgtcaccaccctgccctttttctttaaaaccgaaaagattacttcgcgttatgcaggcttcctcgctcactgactcgctgcgctcggtcgttcggctgcggcgagcggtatcagctcactcaaaggcggtaatacggttatccacagaatcaggggataacgcaggaaagaacatgtgagcaaaaggccagcaaaaggccaggaaccgtaaaaaggccgcgttgctggcgtttttccacaggctccgcccccctgacgagcatcacaaaaatcgacgctcaagtcagaggtggcgaaacccgacaggactataaagataccaggcgtttccccctggaagctccctcgtgcgctctcctgttccgaccctgccgcttaccggatacctgtccgcctttctcccttcgggaagcgtggcgctttctcatagctcacgctgtaggtatctcagttcggtgtaggtcgttcgctccaagctgggctgtgtgcacgaaccccccgttcagcccgaccgctgcgccttatccggtaactatcgtcttgagtccaacccggtaagacacgacttatcgccactggcagcagccactggtaacaggattagcagagcgaggtatgtaggcggtgctacagagttcttgaagtggtggcctaactacggctacactagaagaacagtatttggtatctgcgctctgctgaagccagttaccttcggaaaaagagttggtagctcttgatccggcaaacaaaccaccgctggtagcggtggtttttttgtttgcaagcagcagattacgcgcagaaaaaaaggatctcaagaagatcctttgatcttttctacggggtctgacgctcagtggaacgaaaactcacgttaagggattttggtcatgagattatcaaaaaggatcttcacctagatccttttaaattaaaaatgaagttttaaatcaatctaaagtatatatgagtaaacttggtctgacagctcgaggcttggattctcaccaataaaaaacgcccggcggcaaccgagcgttctgaacaaatccagatggagttctgaggtcattactggatctatcaacaggagtccaagcgagctcgatatcaaattacgccccgccctgccactcgtcgcagtactgttgtaattcattaagcattctgccgacatggaagccatcacaaacggcatgatgaacctgaatcgccagcggcatcagcaccttgtcgccttgcgtataatatttgcccatggtgaaaacgggggcgaagaagttgtccatattggccacgtttaaatcaaaactggtgaaactcacccagggattggctgatacgaaaaacatattctcaataaaccctttagggaaataggccaggttttcaccgtaacacgccacatcttgcgaatatatgtgtagaaactgccggaaatcgtcgtggtattcactccagagtgatgaaaacgtttcagtttgctcatggaaaacggtgtaacaagggtgaacactatcccatatcaccagctcaccgtctttcattgccatacgaaattccggatgagcattcatcaggcgggcaagaatgtgaataaaggccggataaaacttgtgcttatttttctttacggtctttaaaaaggccgtaatatccagctgaacggtctggttataggtacattgagcaactgactgaaatgcctcaaaatgttctttacgatgccattgggatatatcaacggtggtatatccagtgatttttttctccattttagcttccttagctcctgaaaatctcgataactcaaaaaatacgcccggtagtgatcttatttcattatggtgaaagttggaacctcttacgtgcccgatcaactcgagtgccacctgacgtctaagaaaccattattatcatgacattaacctataaaaataggcgtatcacgaggcagaatttcagataaaaaaaatccttagctttcgctaaggatgatttctggaattcgcggccgcttctagagcgatgagtggtctcg

SEQ ID NO: 19 - DNA, 3489 bp, Artificial Sequence
  Plasmid pUPD2-CsUGT2
aatgttgaacggcaacaaatgccacatcctcctcctcccctgtccagcacaaggccatatcaaccccattctccaattcggcaagcgactggcctctcacaacctcctcaccacactcgtcaacacccggttcctctccaactcgaccaaatccgaacccggtccggtcaacatccagtgcatatccgacggattcgatcccggtgggatgaatgcagcacctagtcgtcgggcctatttcgaccgacctcagagtcggtcgggtcagaaacatgttggcctcatcgagtcactccggtccagaggccgacccggcgcatgttttggtctacgacccgttcccctctgggcaatgaacgtagccgagcggtccgggctgcggtcggtcgcattctttactcagccgtgtgcagtggacacaatctaccgccacgtgtgggagggacgaattaaggttccggttgccgagccggtccggttgcctggattgcccccactcgagcctagtgatctgccgtgcgttcgtaacggattcggacgagtcgttaacccggatctcttgccacttcgagtgaatcagcacaaaaatttggacaaagctgacatgatggggaggaactccatatacgagctagaggcggatttgttggatgggtcccgattaccattaccggtgaagtcgattgggccgaccgtgccgtctacttatctcgacaaccgaatcccgtcggattcacactatggattcaatctatacacccctgacactactccctacttggactggctcgactccaaggccccgaactctgtcatctatgtctcatttggtagtttgtccagtctgagccctgatcaaaccaatgagattgcgtcgggtctgatcgccaccaacaaaagctttatttgggtggtacgcacttcggagttagccaaactccctgccaacttcacccaagagaatgcgagccgtgggctggttgtgacctggtgcgaccaactcgatctcctcgcacacgttgcgaccggttgcttcgtgactcactgcggatggaactcgactatggaaggtgtcgcacttggtgtgccgatggtgggagtgccgcagtggtcggaccagcctatgaatgccaagtatgtagaggatgtgtggaaggtcggcgtgagggcgaagacttatgggaaggattttgtgagaggggaggagttcaaaagatgtgtggaggaggtgatggatggagagaggagtggaaagattagagagaatgccgcaaggtggtgtaagttggccaaggactctgttagtgagggtgggagttctgacaagtgtatcaaggagttcatacatcagtgttgcaatgactccaaaatttccttagtttaagctttgagaccactcatcgcgactagtagcggccgctgcagtccggcaaaaaagggcaaggtgtcaccaccctgccctttttctttaaaaccgaaaagattacttcgcgttatgcaggcttcctcgctcactgactcgctgcgctcggtcgttcggctgcggcgagcggtatcagctcactcaaaggcggtaatacggttatccacagaatcaggggataacgcaggaaagaacatgtgagcaaaaggccagcaaaaggccaggaaccgtaaaaaggccgcgttgctggcgtttttccacaggctccgcccccctgacgagcatcacaaaaatcgacgctcaagtcagaggtggcgaaacccgacaggactataaagataccaggcgtttccccctggaagctccctcgtgcgctctcctgttccgaccctgccgcttaccggatacctgtccgcctttctcccttcgggaagcgtggcgctttctcatagctcacgctgtaggtatctcagttcggtgtaggtcgttcgctccaagctgggctgtgtgcacgaaccccccgttcagcccgaccgctgcgccttatccggtaactatcgtcttgagtccaacccggtaagacacgacttatcgccactggcagcagccactggtaacaggattagcagagcgaggtatgtaggcggtgctacagagttcttgaagtggtggcctaactacggctacactagaagaacagtatttggtatctgcgctctgctgaagccagttaccttcggaaaaagagttggtagctcttgatccggcaaacaaaccaccgctggtagcggtggtttttttgtttgcaagcagcagattacgcgcagaaaaaaaggatctcaagaagatcctttgatcttttctacggggtctgacgctcagtggaacgaaaactcacgttaagggattttggtcatgagattatcaaaaaggatcttcacctagatccttttaaattaaaaatgaagttttaaatcaatctaaagtatatatgagtaaacttggtctgacagctcgaggcttggattctcaccaataaaaaacgcccggcggcaaccgagcgttctgaacaaatccagatggagttctgaggtcattactggatctatcaacaggagtccaagcgagctcgatatcaaattacgccccgccctgccactcgtcgcagtactgttgtaattcattaagcattctgccgacatggaagccatcacaaacggcatgatgaacctgaatcgccagcggcatcagcaccttgtcgccttgcgtataatatttgcccatggtgaaaacgggggcgaagaagttgtccatattggccacgtttaaatcaaaactggtgaaactcacccagggattggctgatacgaaaaacatattctcaataaaccctttagggaaataggccaggttttcaccgtaacacgccacatcttgcgaatatatgtgtagaaactgccggaaatcgtcgtggtattcactccagagtgatgaaaacgtttcagtttgctcatggaaaacggtgtaacaagggtgaacactatcccatatcaccagctcaccgtctttcattgccatacgaaattccggatgagcattcatcaggcgggcaagaatgtgaataaaggccggataaaacttgtgcttatttttctttacggtctttaaaaaggccgtaatatccagctgaacggtctggttataggtacattgagcaactgactgaaatgcctcaaaatgttctttacgatgccattgggatatatcaacggtggtatatccagtgatttttttctccattttagcttccttagctcctgaaaatctcgataactcaaaaaatacgcccggtagtgatcttatttcattatggtgaaagttggaacctcttacgtgcccgatcaactcgagtgccacctgacgtctaagaaaccattattatcatgacattaacctataaaaataggcgtatcacgaggcagaatttcagataaaaaaaatccttagctttcgctaaggatgatttctggaattcgcggccgcttctagagcgatgagtggtctcg

SEQ ID NO: 20 - DNA, 3654 bp, Artificial Sequence
  Plasmid pUPD2-UGT709
aatggctgagaaagaagcaaatacccatgtcgtcctcttccccttgccaggccaagggcacatcggctcaatgttgaaactggcacagcttctttccaccgccggattctacgtcactttcgtccacaccgaacgcaactaccgtcgctacctcctcacctccacgtccttccacgtccccaagttccggttccgcaccatccccgacggttttcccgacgacgattcccgctcgcccctcccttttctcgagctccaagagtcgctggacacgaaatgtcgggggcattatcgggaattgttggtcgctgtcgacgaccaagaagagtggcccccagtcacttgtgtcgtggctgatcaagctcttccactctcactcgaagttcccgacgagttggggattcctgtaatgatactcgcaccacacagtgcgtgcagtatattgacgagttattcgattccggagcttataaggggaggtgaactccctatcccagatggggccaatatggatgaactattacaaggcgtactgggattggaaggtatcgtgaggcgtagggatatgtccatcagaagcgccaagtccatccaagatccatttcttcaattcgaagtgaaaatgagcaaaaacttgcccagaggaagagctctcatcctgaacactacagaatcgatagactctctttctttgcgacacattcggtcgatctgtcccactacctacgcactcgggcccttccacgtccttctcaggaacataaaagacgagtcccactccgcaagcctttccgaagaggacaggtcctgcatcgcctggctggactcgaaaccgaacaagtccgcggtctacgtgagtttcggtagcctcgccgccatggcgagagaagcatttcttgagtttcagcagggattgctcgacagcgggtattacttcttgtgggtgatccggcccgatatggtggaaggggggctggaagagagcgagctgaccgcgagcgaacaacgctactttgtgaagtgggccccacaggaggaggttcttgcgcacccggcggtagggtgtttcttgacgcacagcggttggaactctacgttggagagtatctttgcgggagtgccgatgatatgttggcctttctttgcggaccagctgattaacagtaggtttgcgagcgaggtgtggaaaattgccttggatatgaaggatttgtgcggaaggagccacgtggagaggatggtgaaggaagttatgagtggagagaaaggcgaagagctaaggaattctagctgcgagatggcagatagggtgaagaagagtgcagaggaaggtggctcttcctacgccaacttcaaagagttggttggacatatcaaatctttgagcttaccagcagaaagaggagaaaatggtggtgaaggaatgagtgtacaagcgccgagtaaacttttcctcctcaacgctgaggacggaaaacatgtccttaaaagtgacgaaccgtcggaacaaaggggtccacaatttaatccaaattttcttcggacctgagctttgagaccactcatcgcgactagtagcggccgctgcagtccggcaaaaaagggcaaggtgtcaccaccctgccctttttctttaaaaccgaaaagattacttcgcgttatgcaggcttcctcgctcactgactcgctgcgctcggtcgttcggctgcggcgagcggtatcagctcactcaaaggcggtaatacggttatccacagaatcaggggataacgcaggaaagaacatgtgagcaaaaggccagcaaaaggccaggaaccgtaaaaaggccgcgttgctggcgtttttccacaggctccgcccccctgacgagcatcacaaaaatcgacgctcaagtcagaggtggcgaaacccgacaggactataaagataccaggcgtttccccctggaagctccctcgtgcgctctcctgttccgaccctgccgcttaccggatacctgtccgcctttctcccttcgggaagcgtggcgctttctcatagctcacgctgtaggtatctcagttcggtgtaggtcgttcgctccaagctgggctgtgtgcacgaaccccccgttcagcccgaccgctgcgccttatccggtaactatcgtcttgagtccaacccggtaagacacgacttatcgccactggcagcagccactggtaacaggattagcagagcgaggtatgtaggcggtgctacagagttcttgaagtggtggcctaactacggctacactagaagaacagtatttggtatctgcgctctgctgaagccagttaccttcggaaaaagagttggtagctcttgatccggcaaacaaaccaccgctggtagcggtggtttttttgtttgcaagcagcagattacgcgcagaaaaaaaggatctcaagaagatcctttgatcttttctacggggtctgacgctcagtggaacgaaaactcacgttaagggattttggtcatgagattatcaaaaaggatcttcacctagatccttttaaattaaaaatgaagttttaaatcaatctaaagtatatatgagtaaacttggtctgacagctcgaggcttggattctcaccaataaaaaacgcccggcggcaaccgagcgttctgaacaaatccagatggagttctgaggtcattactggatctatcaacaggagtccaagcgagctcgatatcaaattacgccccgccctgccactcgtcgcagtactgttgtaattcattaagcattctgccgacatggaagccatcacaaacggcatgatgaacctgaatcgccagcggcatcagcaccttgtcgccttgcgtataatatttgcccatggtgaaaacgggggcgaagaagttgtccatattggccacgtttaaatcaaaactggtgaaactcacccagggattggctgatacgaaaaacatattctcaataaaccctttagggaaataggccaggttttcaccgtaacacgccacatcttgcgaatatatgtgtagaaactgccggaaatcgtcgtggtattcactccagagtgatgaaaacgtttcagtttgctcatggaaaacggtgtaacaagggtgaacactatcccatatcaccagctcaccgtctttcattgccatacgaaattccggatgagcattcatcaggcgggcaagaatgtgaataaaggccggataaaacttgtgcttatttttctttacggtctttaaaaaggccgtaatatccagctgaacggtctggttataggtacattgagcaactgactgaaatgcctcaaaatgttctttacgatgccattgggatatatcaacggtggtatatccagtgatttttttctccattttagcttccttagctcctgaaaatctcgataactcaaaaaatacgcccggtagtgatcttatttcattatggtgaaagttggaacctcttacgtgcccgatcaactcgagtgccacctgacgtctaagaaaccattattatcatgacattaacctataaaaataggcgtatcacgaggcagaatttcagataaaaaaaatccttagctttcgctaaggatgatttctggaattcgcggccgcttctagagcgatgagtggtctcg

SEQ ID NO: 21 - DNA, 17969 bp, Artificial Sequence
  DNA construct O1= pDGB3alpha1[p35S:UGT2:T35S-p35S:UGT709G1:T35S-pE8:CCD2L:T35S-pNos :Hyg:T35S
ggagactagagccaagctgatctcctttgccccggagatcaccatggacgactttctctatctctacgatctaggaagaaagttcgacggagaaggtgacgataccatgttcaccaccgataatgagaagattagcctcttcaatttcagaaagaatgctgacccacagatggttagagaggcctacgcggcaggtctgatcaagacgatctacccgagtaataatctccaggagatcaaataccttcccaagaaggttaaagatgcagtcaaaagattcaggactaactgcatcaagaacacagagaaagatatatttctcaagatcagaagtactattccagtatggacgattcaaggcttgcttcataaaccaaggcaagtaatagagattggagtctctaagaaagtagttcctactgaatcaaaggccatggagtcaaaaattcagatcgaggatctaacagaactcgccgtgaagactggcgaacagttcatacagagtcttttacgactcaatgacaagaagaaaatcttcgtcaacatggtggagcacgacactctcgtctactccaagaatatcaaagatacagtctcagaagaccaaagggctattgagacttttcaacaaagggtaatatcgggaaacctcctcggattccattgcccagctatctgtcacttcatcaaaaggacagtagaaaaggaaggtggcacctacaaatgccatcattgcgataaaggaaaggctatcgttcaagatgcctctgccgacagtggtcccaaagatggacccccacccacgaggagcatcgtggaaaaagaagacgttccaaccacgtcttcaaagcaagtggattgatgtgatatctccactgacgtaagggatgacgcacaatcccactatccttcgcaagacccttcctctatataaggaagttcatttcatttggagaggactccggtatttttacaacaataccacaacaaaacaaacaacaaacaacattacaatttactattctagtcgaaatgttgaacggcaacaaatgccacatcctcctcctcccctgtccagcacaaggccatatcaaccccattctccaattcggcaagcgactggcctctcacaacctcctcaccacactcgtcaacacccggttcctctccaactcgaccaaatccgaacccggtccggtcaacatccagtgcatatccgacggattcgatcccggtgggatgaatgcagcacctagtcgtcgggcctatttcgaccgacctcagagtcggtcgggtcagaaacatgttggcctcatcgagtcactccggtccagaggccgacccggcgcatgttttggtctacgacccgttcccctctgggcaatgaacgtagccgagcggtccgggctgcggtcggtcgcattctttactcagccgtgtgcagtggacacaatctaccgccacgtgtgggagggacgaattaaggttccggttgccgagccggtccggttgcctggattgcccccactcgagcctagtgatctgccgtgcgttcgtaacggattcggacgagtcgttaacccggatctcttgccacttcgagtgaatcagcacaaaaatttggacaaagctgacatgatggggaggaactccatatacgagctagaggcggatttgttggatgggtcccgattaccattaccggtgaagtcgattgggccgaccgtgccgtctacttatctcgacaaccgaatcccgtcggattcacactatggattcaatctatacacccctgacactactccctacttggactggctcgactccaaggccccgaactctgtcatctatgtctcatttggtagtttgtccagtctgagccctgatcaaaccaatgagattgcgtcgggtctgatcgccaccaacaaaagctttatttgggtggtacgcacttcggagttagccaaactccctgccaacttcacccaagagaatgcgagccgtgggctggttgtgacctggtgcgaccaactcgatctcctcgcacacgttgcgaccggttgcttcgtgactcactgcggatggaactcgactatggaaggtgtcgcacttggtgtgccgatggtgggagtgccgcagtggtcggaccagcctatgaatgccaagtatgtagaggatgtgtggaaggtcggcgtgagggcgaagacttatgggaaggattttgtgagaggggaggagttcaaaagatgtgtggaggaggtgatggatggagagaggagtggaaagattagagagaatgccgcaaggtggtgtaagttggccaaggactctgttagtgagggtgggagttctgacaagtgtatcaaggagttcatacatcagtgttgcaatgactccaaaatttccttagtttaagcttcggccatgctagagtccgcaaaaatcaccagtctctctctacaaatctatctctctctatttttctccagaataatgtgtgagtagttcccagataagggaattagggttcttatagggtttcgctcatgtgttgagcatataagaaacccttagtatgtatttgtatttgtaaaatacttctatcaataaaatttctaattcctaaaaccaaaatccagtgacctcgctgtcaggagactagagccaagctgatctcctttgccccggagatcaccatggacgactttctctatctctacgatctaggaagaaagttcgacggagaaggtgacgataccatgttcaccaccgataatgagaagattagcctcttcaatttcagaaagaatgctgacccacagatggttagagaggcctacgcggcaggtctgatcaagacgatctacccgagtaataatctccaggagatcaaataccttcccaagaaggttaaagatgcagtcaaaagattcaggactaactgcatcaagaacacagagaaagatatatttctcaagatcagaagtactattccagtatggacgattcaaggcttgcttcataaaccaaggcaagtaatagagattggagtctctaagaaagtagttcctactgaatcaaaggccatggagtcaaaaattcagatcgaggatctaacagaactcgccgtgaagactggcgaacagttcatacagagtcttttacgactcaatgacaagaagaaaatcttcgtcaacatggtggagcacgacactctcgtctactccaagaatatcaaagatacagtctcagaagaccaaagggctattgagacttttcaacaaagggtaatatcgggaaacctcctcggattccattgcccagctatctgtcacttcatcaaaaggacagtagaaaaggaaggtggcacctacaaatgccatcattgcgataaaggaaaggctatcgttcaagatgcctctgccgacagtggtcccaaagatggacccccacccacgaggagcatcgtggaaaaagaagacgttccaaccacgtcttcaaagcaagtggattgatgtgatatctccactgacgtaagggatgacgcacaatcccactatccttcgcaagacccttcctctatataaggaagttcatttcatttggagaggactccggtatttttacaacaataccacaacaaaacaaacaacaaacaacattacaatttactattctagtcgaaatggctgagaaagaagcaaatacccatgtcgtcctcttccccttgccaggccaagggcacatcggctcaatgttgaaactggcacagcttctttccaccgccggattctacgtcactttcgtccacaccgaacgcaactaccgtcgctacctcctcacctccacgtccttccacgtccccaagttccggttccgcaccatccccgacggttttcccgacgacgattcccgctcgcccctcccttttctcgagctccaagagtcgctggacacgaaatgtcgggggcattatcgggaattgttggtcgctgtcgacgaccaagaagagtggcccccagtcacttgtgtcgtggctgatcaagctcttccactctcactcgaagttcccgacgagttggggattcctgtaatgatactcgcaccacacagtgcgtgcagtatattgacgagttattcgattccggagcttataaggggaggtgaactccctatcccagatggggccaatatggatgaactattacaaggcgtactgggattggaaggtatcgtgaggcgtagggatatgtccatcagaagcgccaagtccatccaagatccatttcttcaattcgaagtgaaaatgagcaaaaacttgcccagaggaagagctctcatcctgaacactacagaatcgatagactctctttctttgcgacacattcggtcgatctgtcccactacctacgcactcgggcccttccacgtccttctcaggaacataaaagacgagtcccactccgcaagcctttccgaagaggacaggtcctgcatcgcctggctggactcgaaaccgaacaagtccgcggtctacgtgagtttcggtagcctcgccgccatggcgagagaagcatttcttgagtttcagcagggattgctcgacagcgggtattacttcttgtgggtgatccggcccgatatggtggaaggggggctggaagagagcgagctgaccgcgagcgaacaacgctactttgtgaagtgggccccacaggaggaggttcttgcgcacccggcggtagggtgtttcttgacgcacagcggttggaactctacgttggagagtatctttgcgggagtgccgatgatatgttggcctttctttgcggaccagctgattaacagtaggtttgcgagcgaggtgtggaaaattgccttggatatgaaggatttgtgcggaaggagccacgtggagaggatggtgaaggaagttatgagtggagagaaaggcgaagagctaaggaattctagctgcgagatggcagatagggtgaagaagagtgcagaggaaggtggctcttcctacgccaacttcaaagagttggttggacatatcaaatctttgagcttaccagcagaaagaggagaaaatggtggtgaaggaatgagtgtacaagcgccgagtaaacttttcctcctcaacgctgaggacggaaaacatgtccttaaaagtgacgaaccgtcggaacaaaggggtccacaatttaatccaaattttcttcggacctgagcttcggccatgctagagtccgcaaaaatcaccagtctctctctacaaatctatctctctctatttttctccagaataatgtgtgagtagttcccagataagggaattagggttcttatagggtttcgctcatgtgttgagcatataagaaacccttagtatgtatttgtatttgtaaaatacttctatcaataaaatttctaattcctaaaaccaaaatccagtgacctcgctgtcaggagagcgcgagtcggtcccattattgaagcatttatcagggttattgtctcatgagcggatacatatttgaatgtatttagaaaaataaacaaataggggttccgcgcacatttccccgaaaagtgccacctgacgtctaagaaaccattattatcatgacattaacctataaaaataggcgtatcacgaggccctttcgtcttcaagaattagcttggcaattcccgatctagtaacatagatgacaccghgcgcgataatttatcctagtttgcgcgctatattttgttttctatcgcgtattaaatgtataattgcgggactctaatcataaaaacccatctcataaataacgtcatgcattacatgttaattattacatgcttaacgtaattcaacagaaattatatgataatcgtcgcaagaccggcaacaggattcaatcttaagaaactttattgccaaatgtttgaacgatcgggatcgaagatccattccaagctcattcctttgccctcggacgagtgctggggcgtcggtttccactatcggcgagtacttctacacagccatcggtccagacggccgcgcttctgcgggcgatttgtgtacgcccgacagtcccggctccggatcggacgattgcgtcgcatcgaccctgcgcccaagctgcatcatcgaaattgccgtcaaccaagctctgatagagttggtcaagaccaatgcggagcatatacgcccggagtcgtggcgatcctgcaagctccggatgcctccgctcgaagtagcgcgtctgctgctccatacaagccaaccacggcctccagaagaagatgttggcgacctcgtattgggaatccccgaacattgcctcgctccagtcaatgaccgctgttatgcggccattgtccgtcaggacattgttggagccgaaatccgcgtgcacgaggtgccggacttcggggcagtcctcggcccaaagcatcagctcatcgagagcctgcgcgacggacgcactgacggtgtcgtccatcacagtttgccagtgatacacatggggatcagcaatcgcgcatatgaaatcacgccatgtagtgtattgaccgattccttgcggtccgaatgggccgaacccgctcgtctggctaagatcggccgcagcgatcgcatccatggcctccgcgaccggctgcagaacagcgggcagttcggtttcaggcaggtcttgcaacgtgacaccctgtgcacggcgggagatgcaataggtcaggctctcgctgaattccccaatgtcaagcacttccggaatcgggagcgcggccgatgcaaagtgccgataaacataacgatctttgtagaaaccatcggcgcagctatttacccgcaggacatatccacgccctcctacatcgaagctgaaagcacgagattcttcgccctccgagagctgcatcaggtcggacacgctgtcgaacttttcgatcagaaacttctcgacagacgtcgcggtgagttcaggctttttcattgcctcgatcgagttgagagtgaatatgagactctaattggataccgaggggaatttatggaacgtcagtggagcatttttgacaagaaatatttgctagctgatagtgaccttaggcgacttttgaacgcgcaataatggtttctgacgtatgtgcttagctcattaaactccagaaacccgcggctcagtggctccttcaacgttgcggttctgtcagttccaaacgtaaaacggcttgtcccgcgtcatcggcgggggtcataccgtgactcccttaattctcatgtatctccgtcaggagtccctaatgatattgttcacgtaattaagttttgtggaagtgagagagtccaattttgataagaaaagagtcagaaaacgtaatattttaaaagtctaaatctttctacaaataagagcaaatttatttattttttaatccaataaatattaatggaggacaaattcaattcacttggttgtaaaataaacttaaaccaataaccaaagaactaataaatcctgaagtggaattattaaggataaatgtacatagacaatgaagaaataataggttcgatgaattaataataattaaggatgttacaatcatcatgtgccaagtatatacacaatattctatgggatttataatttcgttacttcacttaacttttgcgtaaataaaacgaattatctgatattttataataaaacagttataagaaccatcatttttaacaacatagatatattatttctaatagtttaatgatacttttaaatcttttaaattttatgtttcttttagaaaataaaaattcaaaaaattaaatatatttacaaaaactacaatcaaacacaacttcatatattaaaagcaaaatatattttgaaaatttcaagtgtcctaacaaataagacaagaggaaaatgtacgatgagagacataaagagaactaataattgaggagtcctataatatataataaagtttattagtaaacttaattattaaggactcctaaaatatatgataggagaaaatgaatggtgagagatattggaaaacttaataattaaggattttaaaatatatggtaaaagataggcaaagtatccattatccccttttaacttgaagtctactaggcgcatgtgaaagttgattttttgtcacgtcatatagctataacgtaaaaaaagaaagtaaaatttttaattttttttaatatatgacatattttaaacgaaatataggacaaaatgtaaatgaatagtaaaggaaacaaagattaatacttactttgtaagaatttaagataaatttaaaatttaatagatcaactttacgtctagaaagacccatatctagaaggaatttcacgaaatcggcccttattcgaaaataacttttaaataatgaattttaaattttaagaaataatatccaatgaataaatgacatgtagcattttacctaaatatttcaactattttaatccaatattaatttgttttattcccaacaatagaaagtcttgtgcagacatttaatctgacttttccagtactaaatattaattttctgaagattttcgggtttagtccacaagttttagtgagaagttttgctcaaattttaggtgagaaggtttgatatttatcttttgttaaattaatttatctaggtgactattatttatttaagtagaaattcatatcattacttttgccaacttgtagtcataataggagtaggtgtatatgatgaaggaataaacaagttcagtgaagtgattaaaataaaatataatttaggtgtacatcaaataaaaaccttaaagtttagaaaggcaccgaataattttgcatagaagatattagtaaatttataaaaataaaagaaatgtagttgtcaagttgtcttcttttttttggataaaaatagcagttggcttatgtcattcttttacaacctccatgccacttgtccaattgttgacacttaactaattagtttgattcatgtatgaatactaaataattttttaggactgactcaaatatttttatattatcatagtaatatttatctaatttttaggaccacttattactaaataataaattaactacaactatattattgttgtgaaacaacaacgttttggttgttatgatgaaacgtacactatatcagtatgaaaaattcaaaacgattagtataaattatattgaaaatttgatatttttctattcttaatcagacgtattgggtttcatattttaaaaagggactaaacttagaagagaagtttgtttgaaactacttttgtctctttcttgttcccatttctctcttagatttcaaaaagtgaactactttatctccttctttgttcacattttattttattctattataaatatggcatcctcatattgagatttttagaaattattctaatcattcacagtgcaaaagaagaatggaatctcctgctactaaattacctgcacctctgctgatgttatcttcttctccattccttctcccttctcctaataagagctcctccatcttccttccacgtaaattagggccgctacctccaaaatattattattacaattgctgccatcctaagagtagatcaatctcagtagtatcaatggcaaataaggaggaggcagagacaagtaagaagaagcccaaaccattaaaagtactaattaccaaagtggatccgaagccgaggaagggcatggcatccgtcgcagtggacttactcgagaaggcctttgtatacctattgtccggaaattctgcagctgatcgtagtagtagtagtggtcgtcgtcgtcgtaaagagcattactacctctccggcaattatgcgcccgtcggacacgaaaccccgccctccgaccacctccccattcatggatcccttcctgaatgcttgaatggagtgtttctgagagttggtcctaaccccaagtttgctcccgtagccggatacaattgggtcgatggagatggaatgattcatggattgcgtattaaagatggaaaagcaacttatctatctcgatatattaaaacgtcacggtttaaacaagaagaatattttggaagagcaaaatttatgaagattggagatctaaggggattgcttgggttctttacgatcttaatactagtacttcgaacaacattgaaagtaatagacatttcatatggaagagggacgggtaatacagctcttgtgtatcataatggcttactattggctctatcagaagaagataaaccttatgttgttaaagttttagaagatggagacttgcaaactcttgggatattggattatgacaagaaattgtcacatccattcaccgctcatccaaagatcgatccgttaactgatgagatgtttacctttggatattccatctcgcctccgtatcttacttatcgagtcatttccaaggatggagtgatgcaagatccagtgcaaatctcaattacatcccctaccataatgcatgattttgctattactgaaaattatgccatcttcatggacctgcccttgtatttccaaccagaggaaatggtaaaggggaaatttgtctcttcatttcaccctacaaaaagagctcgtatcggtgtgcttccacgatatgcaaaagacgagcatccaattcgatggttcgatcttccaagttgcttcatgactcataatgcaaatgcttgggaagagaatgatgaagttgtgctattcacatgtcgccttgagagtcctgatcttgacatgcttagtggacctgcggaagaagagattgggaattcaaaaagtgagctttacgaaatgaggttcaatttgaaaactggaattacttcacaaaagcaactatctgtacctagtgttgattttcctcggatcaaccaaagttatactggcaggaaacagcaatatgtttattgtactcttggcaacaccaagattaagggcattgtgaagtttgatctgcaaattgaaccagaagccggaaagacaatgcttgaagttggaggaaatgtacaaggcatctttgagttgggacctagaagatatggttcagaggcaatatttgtgccatgccaacctggcatcaaatctgatgaggatgacggttacttgatattctttgtacacgacgaaaacaatgggaaatctgaggtcaatgtcatcgatgcaaagacaatgtctgcagaacctgtggctgttgtggaacttccaagcagggttccatatggattccatgccttgtttctgaatgaggaagaacttcagaagcaccaagcagagacatgagcttcggccatgctagagtccgcaaaaatcaccagtctctctctacaaatctatctctctctatttttctccagaataatgtgtgagtagttcccagataagggaattagggttcttatagggtttcgctcatgtgttgagcatataagaaacccttagtatgtatttgtatttgtaaaatacttctatcaataaaatttctaattcctaaaaccaaaatccagtgacctcgctgtcatgagacgaattctgacaggatatattggcgggtaaacctaagagaaaagagcgtttattagaataatcggatatttaaaagggcgtgaaaaggtttatccgttcgtccatttgtatgtgcatgccaaccacagggttcccctcgggatcaaagtactttgatccaacccctccgctgctatagtgcagtcggcttctgacgttcagtgcagccgtcatctgaaaacgacatgtcgcacaagtcctaagttacgcgacaggctgccgccctgcccttttcctggcgttttcttgtcgcgtgttttagtcgcataaagtagaatacttgcgactagaaccggagacattacgccatgaacaagagcgccgccgctggcctgctgggctatgcccgcgtcagcaccgacgaccaggacttgaccaaccaacgggccgaactgcacgcggccggctgcaccaagctgttttccgagaagatcaccggcaccaggcgcgaccgcccggagctggccaggatgcttgaccacctacgccctggcgacgttgtgacagtgaccaggctagaccgcctggcccgcagcacccgcgacctactggacattgccgagcgcatccaggaggccggcgcgggcctgcgtagcctggcagagccgtgggccgacaccaccacgccggccggccgcatggtgttgaccgtgttcgccggcattgccgagttcgagcgttccctaatcatcgaccgcacccggagcgggcgcgaggccgccaaggcccgaggcgtgaagtttggcccccgccctaccctcaccccggcacagatcgcgcacgcccgcgagctgatcgaccaggaaggccgcaccgtgaaagaggcggctgcactgcttggcgtgcatcgctcgaccctgtaccgcgcacttgagcgcagcgaggaagtgacgcccaccgaggccaggcggcgcggtgccttccgtgaggacgcattgaccgaggccgacgccctggcggccgccgagaatgaacgccaagaggaacaagcatgaaaccgcaccaggacggccaggacgaaccgtttttcattaccgaagagatcgaggcggagatgatcgcggccgggtacgtgttcgagccgcccgcgcacctctcaaccgtgcggctgcatgaaatcctggccggtttgtctgatgccaagctggcggcctggccggccagcttggccgctgaagaaaccgagcgccgccgtctaaaaaggtgatgtgtatttgagtaaaacagcttgcgtcatgcggtcgctgcgtatatgatccgatgagtaaataaacaaatacgcaaggggaacgcatgaaggttatcgctgtacttaaccagaaaggcgggtcaggcaagacgaccatcggaacccatctagcccgcgccctgcaactcgccggggccgatgttctgttagtcgattccgatccccagggcagtgcccgcgattgggcggccgtgcgggaagatcaaccgctaaccgttgtcggcatcgaccgcccgacgattgaccgcgacgtgaaggccatcggccggcgcgacttcgtagtgatcgacggagcgccccaggcggcggacttggctgtgtccgcgatcaaggcagccgacttcgtgctgattccggtgcagccaagcccttacgacatatgggccaccgccgacctggtggagctggttaagcagcgcattgaggtcacggatggaaggctacaagcggcctttgtcgtgtcgcgggcgatcaaaggcacgcgcatcggcggtgaggttgccgaggcgctggccgggtacgagctgcccattcttgagtcccgtatcacgcagcgcgtgagctacccaggcactgccgccgccggcacaaccgttcttgaatcagaacccgagggcgacgctgcccgcgaggtccaggcgctggccgctgaaattaaatcaaaactcatttgagttaatgaggtaaagagaaaatgagcaaaagcacaaacacgctaagtgccggccgtccgagcgcacgcagcagcaaggctgcaacgttggccagcctggcagacacgccagccatgaagcgggtcaactttcagttgccggcggaggatcacaccaagctgaagatgtacgcggtacgccaaggcaagaccattaccgagctgctatctgaatagatcgcgcagctaccagagtaaatgagcaaatgaataaatgagtagatgaattttagcggctaaaggaggcggcatggaaaatcaagaacaaccaggcaccgacgccgtggaatgccccatgtgtggaggaacgggcggttggccaggcgtaagcggctgggttgtctgccggccctgcaatggcactggaacccccaagcccgaggaatcggcgtgacggtcgcaaaccatccggcccggtacaaatcggcgcggcgctgggtgatgacctggtggagaagttgaaggccgcgcaggccgcccagcggcaacgcatcgaggcagaagcacgccccggtgaatcgtggcaagcggccgctgatcgaatccgcaaagaatcccggcaaccgccggcagccggtgcgccgtcgattaggaagccgcccaagggcgacgagcaaccagattttttcgttccgatgctctatgacgtgggcacccgcgatagtcgcagcatcatggacgtggccgttttccgtctgtcgaagcgtgaccgacgagctggcgaggtgatccgctacgagcttccagacgggcacgtagaggtttccgcagggccggccggcatggccagtgtgtgggattacgacctggtactgatggcggtttcccatctaaccgaatccatgaaccgataccgggaagggaagggagacaagcccggccgcgtgttccgtccacacgttgcggacgtactcaagttctgccggcgagccgatggcggaaagcagaaagacgacctggtagaaacctgcattcggttaaacaccacgcacgttgccatgcagcgtacgaagaaggccaagaacggccgcctggtgacggtatccgagggtgaagccttgattagccgctacaagatcgtaaagagcgaaaccgggcggccggagtacatcgagatcgagctagctgattggatgtaccgcgagatcacagaaggcaagaacccggacgtgctgacggttcaccccgattactttttgatcgatcccggcatcggccgttttctctaccgcctggcacgccgcgccgcaggcaaggcagaagccagatggttgttcaagacgatctacgaacgcagtggcagcgccggagagttcaagaagttctgtttcaccgtgcgcaagctgatcgggtcaaatgacctgccggagtacgatttgaaggaggaggcggggcaggctggcccgatcctagtcatgcgctaccgcaacctgatcgagggcgaagcatccgccggttcctaatgtacggagcagatgctagggcaaattgccctagcaggggaaaaaggtcgaaaaggactctttcctgtggatagcacgtacattgggaacccaaagccgtacattgggaaccggaacccgtacattgggaacccaaagccgtacattgggaaccggtcacacatgtaagtgactgatataaaagagaaaaaaggcgatttttccgcctaaaactctttaaaacttattaaaactcttaaaacccgcctggcctgtgcataactgtctggccagcgcacagccgaagagctgcaaaaagcgcctacccttcggtcgctgcgctccctacgccccgccgcttcgcgtcggcctatcgcggccgctggccgctcaaaaatggctggcctacggccaggcaatctaccagggcgcggacaagccgcgccgtcgccactcgaccgccggcgcccacatcaaggcaccctgcctcgcgcgtttcggtgatgacggtgaaaacctctgacacatgcagctcccggtgacggtcacagcttgtctgtaagcggatgccgggagcagacaagcccgtcagggcgcgtcagcgggtgttggcgggtgtcggggcgcagccatgacccagtcacgtagcgatagcggagtgtatactggcttaactatgcggcatcagagcagattgtactgagagtgcaccatatgcggtgtgaaataccgcacagatgcgtaaggagaaaataccgcatcaggcgctcttccgcttcctcgctcactgactcgctgcgctcggtcgttcggctgcggcgagcggtatcagctcactcaaaggcggtaatacggttatccacagaatcaggggataacgcaggaaagaacatgtgagcaaaaggccagcaaaaggccaggaaccgtaaaaaggccgcgttgctggcgtttttccataggctccgcccccctgacgagcatcacaaaaatcgacgctcaagtcagaggtggcgaaacccgacaggactataaagataccaggcgtttccccctggaagctccctcgtgcgctctcctgttccgaccctgccgcttaccggatacctgtccgcctttctcccttcgggaagcgtggcgctttctcatagctcacgctgtaggtatctcagttcggtgtaggtcgttcgctccaagctgggctgtgtgcacgaaccccccgttcagcccgaccgctgcgccttatccggtaactatcgtcttgagtccaacccggtaagacacgacttatcgccactggcagcagccactggtaacaggattagcagagcgaggtatgtaggcggtgctacagagttcttgaagtggtggcctaactacggctacactagaaggacagtatttggtatctgcgctctgctgaagccagttaccttcggaaaaagagttggtagctcttgatccggcaaacaaaccaccgctggtagcggtggtttttttgtttgcaagcagcagattacgcgcagaaaaaaaggatctcaagaagatcctttgatcttttctacggggtctgacgctcagtggaacgaaaactcacgttaagggattttggtcatgcattctaggtgattagaaaaactcatcgagcatcaaatgaaactgcaatttattcatatcaggattatcaataccatatttttgaaaaagccgtttctgtaatgaaggagaaaactcaccgaggcagttccataggatggcaagatcctggtatcggtctgcgattccgactcgtccaacatcaatacaacctattaatttcccctcgtcaaaaataaggttatcaagtgagaaatcaccatgagtgacgactgaatccggtgagaatggcaaaagtttatgcatttctttccagacttgttcaacaggccagccattacgctcgtcatcaaaatcactcgcatcaaccaaaccgttattcattcgtgattgcgcctgagcgagtcgaaatacgcgatcgctgttaaaaggacaattacaaacaggaatcgaatgcaaccggcgcaggaacactgccagcgcatcaacaatattttcacctgaatcaggatattcttctaatacctggaatgctgttttccctgggatcgcagtggtgagtaaccatgcatcatcaggagtacggataaaatgcttgatggtcggaagaggcataaattccgtcagccagtttagtctgaccatctcatctgtaacatcattggcaacgctacctttgccatgtttcagaaacaactctggcgcatcgggcttcccatacaatcggtagattgtcgcacctgattgcccgacattatcgcgagcccatttatacccatataaatcagcatccatgttggaatttaatcgcggccttgagcaagacgtttcccgttgaatatggctcataacagaacttattatttccttcctcttttctacagtatttaaagataccccaagaagctaattataacaagacgaactccaattcactgttccttgcattctaaaaccttaaataccagaaaacagctttttcaaagttgttttcaaagttggcgtataacatagtatcgacggagccgattttgaaaccgcggtgatcacaggcagcaacgctctgtcatcgttacaatcaacatgctaccctccgcgagatcatccgtgtttcaaacccggcagcttagttgccgttcttccgaatagcatcggtaacatgagcaaagtctgccgccttacaacggctctcccgctgacgccgtcccggactgatgggctgcctgtatcgagtggtgattttgtgccgagctgccggtcggggagctgttggctggctggtggcaggatatattgtggtgtaaacataacgaattcgtctca

SEQ ID NO: 22 - DNA, 20976 bp, Artificial Sequence
  DNA construct O2 = pDGB3?1[p2A11:UGT2:T35S-p35S:UGT709G1:T35S-pE8:CCD2L:T35S-pNos:Hy g:T35S]
ggaggtcaaacaattttgaggaattcaatttcatctttaactggtacaataatcattttatcatgaaaataagcagctcaagagaatttttgaagaatcttttatttctttaacatttaaccacatgaatttttaatttttttttgcaatacatttaaaccgaaatggtcaaacgatcaaccaactgatctttattctaataaacttctagtttacatttgcatgtgagtgcatcatcattatcatatttgtacacaacaaacaagaaaaaaatataaacaatattttatttaaatatttatattccactttgactgtagatattaaatcttgtcatcatttatagtctcaatattataatttttttattttttcaaaattcaaaagtttacaattatttttttgaactataatattatccaagatgaacatctcaagaagaaaattattaatattgttatggttaaaattttacatacaatacttgttttttgctttacttttatcttaccgtagatacacaatcgacgataacttagtgatcacacaataataattattttgttcatgacacaatatttataagaaatacttatttctttcttttatccttcagtagttcataataaaaacataccataatatttgtgatgcattcatagtacgtaatgaaatgacaatttatgtcaaattattttcttttatactctcaaacctcccgtaaaggtgagatgagtcatttatccaattatacataaatatgtctttattcatgctctttatcacattctgacacattcacttaatttcaagagtaagcaagcatgataactgaaactatttatgcgtatcttaccttgatatttgacacattacatgacacacctcaacatcactttcaaagattaagcgcaccaccatattatctttctttttttttttatgaaggttttataaaattattaaattaggtccaaaaaattgtttgtcaaataaccttttatactagattgatgacaaaaattacctttacgttttgaaagaccattttaagacctaatctatcagtgactccttaaagttggcacaatatttcacttagacaccctaattgaatgatgttcattttaaacacccaatgtagggttccgctatatcattttgacacatttcttaacatcaacaaaaatatataatgagtatgtgatatactcgcgaatgacgtgaaaaatgaagacatttgttatttgtatcaaagtagttactaaataattaattttgaataaaaataaaagctgaccagtaaatcaataacacataatattttccacctaataattaaaatataaaataaaaaagagccatctcagggtcatctgcccaccattgctatttcaaagaaatttgtacgttagtttatagaaattgatgttaaaattctttcaagaaaaatttatgaatgaatttattctctaatttaaaaatattttctgttatttttgttgaaagaaatttaacttggataaaatggtggttaaaactggaaagaagaaaagagaaaaaataattaaaaatcatttcacgctctaatcaatgagcgtatcacattcattatgttatataagcaaaagtgacaaaacgaaaataatatattacatgaaatgtctaaaataaatatcgtctaattaaaatatctaagtaacatattgtgcctaactttagagggatcatcaataagttaaaccccattttaataactcataattgtcctttttatttaatattgtcacaaatcacaatgataattaacattaatttgtcctttgtgacgtccatattcatgcatttaaccaatcatcttcatttggacttattatcacaattatcccactttcctcacaaaatggagcattcaagtggaatagactacacgatttttaatttcatcaaaaacatctttttgctttattcattattatattgtcgctattgttgaattttatttgccctaaatttcttaccataaatagatttttcttttagaaaaaggagattgactaattcttttcttgtaggaaaaggtttaggactctataaatagagacatattccttctaacttaatcaacatttacaatgtagtcttaaagactttgaaagtttttggttagggggagaaattgtgggtcacaagcttgatacgttatcaattgtgtaaacctcccatgtattctgagtgaatttggttgaggttgtttccctctgtattttgtactctcatatttatagtggattgttcatctctttcgtggacgtaggtcgattgaccgtcgattgaccgaaccacgttaaatctttgtattttttgatatatttctcattatcttcttactcgtgatctttcaaggtttgcattgctatcttccgcgttacaccaacttatttacgatcctaacagctatggtgtggaaacataaatcaaacattttactgatataaacacatctttgattataacatgatagaaatttgagcccaactttttatcatcattatatacaaaaagttctaaattttttttttgatgtagtaaaacttaaatccatagtcttgcccctaaaccaatgacataatatataacccaaaatatactagttttcgccctcgagccctttaaaaagtatagtcaatatttacggtgaccgtgaatttcttaattatgatatataatttaaaagaaatcatgatcacattctactgatgagaacatgtgctaatcaagggaaaacatggatgtgaaaaatactttttgttaaaagtaaaaaaaaatgtgaaattttgttagttatttactacctatacattatttgagcatgtgcaaactttacaaatacctaatagaagattttcacctgcctgtatatatgtaaattaattataatgaacactctcacataaaataattatcagtatatacattaatacttgccctccacaatgaattaaataaaatgtagaacatgatctacacttcaataaaactaagaccataaagaataatttcaaaatatacacatgtcaacaataaattatttgcatattatattaacttactaaacaatctttacttttgaaatataaaaataatcaagttataagtctgctcaaagtaaagcacttgttagactcatctgattttgagaaggtaagcaaattgatggtgcataatagtcacaagtaaaatataaaatagatttcattagtaaaattgttttttactttctttatatataattatcaatatccttcaatggtaggttaattatattgttaacttcttgttgaattaaagcaataagacaagaatattaaagataaaagaacaataaaaatagaaagactaagagataagagttttcttattcttctttcaataagtatcatcaagtgtatacaatataaatttttgtatttttgatctatctatttataatgttatatataagcatacaaaagatcagtcataaatatgactttaatcatgaaaataatgaaagagattatgaaggcgtaaggttactagaataatagtcattaaaaaaaggggttatctttataattgaataattgatgaagtaatggagataattagtgagcataaatttttttaaaaaaatggacatttacactataatattttataacactttcccttaaacatctaggtataaataatgagtcttgtcaaaatcttagtaggaaaaattctgtgaaatttttttagtgaaaacaaatgatataaatatcttgaatactcattatttgttgtctcattaaaaatcttatctgacctataaaataaattatttgctcaactcaaaatagtttttcattctaaaattagtataattattagtgaatatttaattaacataattgtatactaaggggcctataaattggattcttctcaaagaaaaataaaatcaccacacaactttcttcttctgctcatcaattagcaattaatccaaaaccaaatgttgaacggcaacaaatgccacatcctcctcctcccctgtccagcacaaggccatatcaaccccattctccaattcggcaagcgactggcctctcacaacctcctcaccacactcgtcaacacccggttcctctccaactcgaccaaatccgaacccggtccggtcaacatccagtgcatatccgacggattcgatcccggtgggatgaatgcagcacctagtcgtcgggcctatttcgaccgacctcagagtcggtcgggtcagaaacatgttggcctcatcgagtcactccggtccagaggccgacccggcgcatgttttggtctacgacccgttcccctctgggcaatgaacgtagccgagcggtccgggctgcggtcggtcgcattctttactcagccgtgtgcagtggacacaatctaccgccacgtgtgggagggacgaattaaggttccggttgccgagccggtccggttgcctggattgcccccactcgagcctagtgatctgccgtgcgttcgtaacggattcggacgagtcgttaacccggatctcttgccacttcgagtgaatcagcacaaaaatttggacaaagctgacatgatggggaggaactccatatacgagctagaggcggatttgttggatgggtcccgattaccattaccggtgaagtcgattgggccgaccgtgccgtctacttatctcgacaaccgaatcccgtcggattcacactatggattcaatctatacacccctgacactactccctacttggactggctcgactccaaggccccgaactctgtcatctatgtctcatttggtagtttgtccagtctgagccctgatcaaaccaatgagattgcgtcgggtctgatcgccaccaacaaaagctttatttgggtggtacgcacttcggagttagccaaactccctgccaacttcacccaagagaatgcgagccgtgggctggttgtgacctggtgcgaccaactcgatctcctcgcacacgttgcgaccggttgcttcgtgactcactgcggatggaactcgactatggaaggtgtcgcacttggtgtgccgatggtgggagtgccgcagtggtcggaccagcctatgaatgccaagtatgtagaggatgtgtggaaggtcggcgtgagggcgaagacttatgggaaggattttgtgagaggggaggagttcaaaagatgtgtggaggaggtgatggatggagagaggagtggaaagattagagagaatgccgcaaggtggtgtaagttggccaaggactctgttagtgagggtgggagttctgacaagtgtatcaaggagttcatacatcagtgttgcaatgactccaaaatttccttagtttaagcttcggccatgctagagtccgcaaaaatcaccagtctctctctacaaatctatctctctctatttttctccagaataatgtgtgagtagttcccagataagggaattagggttcttatagggtttcgctcatgtgttgagcatataagaaacccttagtatgtatttgtatttgtaaaatacttctatcaataaaatttctaattcctaaaaccaaaatccagtgacctcgctgtcaggagactagagccaagctgatctcctttgccccggagatcaccatggacgactttctctatctctacgatctaggaagaaagttcgacggagaaggtgacgataccatgttcaccaccgataatgagaagattagcctcttcaatttcagaaagaatgctgacccacagatggttagagaggcctacgcggcaggtctgatcaagacgatctacccgagtaataatctccaggagatcaaataccttcccaagaaggttaaagatgcagtcaaaagattcaggactaactgcatcaagaacacagagaaagatatatttctcaagatcagaagtactattccagtatggacgattcaaggcttgcttcataaaccaaggcaagtaatagagattggagtctctaagaaagtagttcctactgaatcaaaggccatggagtcaaaaattcagatcgaggatctaacagaactcgccgtgaagactggcgaacagttcatacagagtcttttacgactcaatgacaagaagaaaatcttcgtcaacatggtggagcacgacactctcgtctactccaagaatatcaaagatacagtctcagaagaccaaagggctattgagacttttcaacaaagggtaatatcgggaaacctcctcggattccattgcccagctatctgtcacttcatcaaaaggacagtagaaaaggaaggtggcacctacaaatgccatcattgcgataaaggaaaggctatcgttcaagatgcctctgccgacagtggtcccaaagatggacccccacccacgaggagcatcgtggaaaaagaagacgttccaaccacgtcttcaaagcaagtggattgatgtgatatctccactgacgtaagggatgacgcacaatcccactatccttcgcaagacccttcctctatataaggaagttcatttcatttggagaggactccggtatttttacaacaataccacaacaaaacaaacaacaaacaacattacaatttactattctagtcgaaatggctgagaaagaagcaaatacccatgtcgtcctcttccccttgccaggccaagggcacatcggctcaatgttgaaactggcacagcttctttccaccgccggattctacgtcactttcgtccacaccgaacgcaactaccgtcgctacctcctcacctccacgtccttccacgtccccaagttccggttccgcaccatccccgacggttttcccgacgacgattcccgctcgcccctcccttttctcgagctccaagagtcgctggacacgaaatgtcgggggcattatcgggaattgttggtcgctgtcgacgaccaagaagagtggcccccagtcacttgtgtcgtggctgatcaagctcttccactctcactcgaagttcccgacgagttggggattcctgtaatgatactcgcaccacacagtgcgtgcagtatattgacgagttattcgattccggagcttataaggggaggtgaactccctatcccagatggggccaatatggatgaactattacaaggcgtactgggattggaaggtatcgtgaggcgtagggatatgtccatcagaagcgccaagtccatccaagatccatttcttcaattcgaagtgaaaatgagcaaaaacttgcccagaggaagagctctcatcctgaacactacagaatcgatagactctctttctttgcgacacattcggtcgatctgtcccactacctacgcactcgggcccttccacgtccttctcaggaacataaaagacgagtcccactccgcaagcctttccgaagaggacaggtcctgcatcgcctggctggactcgaaaccgaacaagtccgcggtctacgtgagtttcggtagcctcgccgccatggcgagagaagcatttcttgagtttcagcagggattgctcgacagcgggtattacttcttgtgggtgatccggcccgatatggtggaaggggggctggaagagagcgagctgaccgcgagcgaacaacgctactttgtgaagtgggccccacaggaggaggttcttgcgcacccggcggtagggtgtttcttgacgcacagcggttggaactctacgttggagagtatctttgcgggagtgccgatgatatgttggcctttctttgcggaccagctgattaacagtaggtttgcgagcgaggtgtggaaaattgccttggatatgaaggatttgtgcggaaggagccacgtggagaggatggtgaaggaagttatgagtggagagaaaggcgaagagctaaggaattctagctgcgagatggcagatagggtgaagaagagtgcagaggaaggtggctcttcctacgccaacttcaaagagttggttggacatatcaaatctttgagcttaccagcagaaagaggagaaaatggtggtgaaggaatgagtgtacaagcgccgagtaaacttttcctcctcaacgctgaggacggaaaacatgtccttaaaagtgacgaaccgtcggaacaaaggggtccacaatttaatccaaattttcttcggacctgagcttcggccatgctagagtccgcaaaaatcaccagtctctctctacaaatctatctctctctatttttctccagaataatgtgtgagtagttcccagataagggaattagggttcttatagggtttcgctcatgtgttgagcatataagaaacccttagtatgtatttgtatttgtaaaatacttctatcaataaaatttctaattcctaaaaccaaaatccagtgacctcgctgtcaggagagcgcgagtcggtcccattattgaagcatttatcagggttattgtctcatgagcggatacatatttgaatgtatttagaaaaataaacaaataggggttccgcgcacatttccccgaaaagtgccacctgacgtctaagaaaccattattatcatgacattaacctataaaaataggcgtatcacgaggccctttcgtcttcaagaattagcttggcaattcccgatctagtaacatagatgacaccghgcgcgataatttatcctagtttgcgcgctatattttgttttctatcgcgtattaaatgtataattgcgggactctaatcataaaaacccatctcataaataacgtcatgcattacatgttaattattacatgcttaacgtaattcaacagaaattatatgataatcgtcgcaagaccggcaacaggattcaatcttaagaaactttattgccaaatgtttgaacgatcgggatcgaagatccattccaagctcattcctttgccctcggacgagtgctggggcgtcggtttccactatcggcgagtacttctacacagccatcggtccagacggccgcgcttctgcgggcgatttgtgtacgcccgacagtcccggctccggatcggacgattgcgtcgcatcgaccctgcgcccaagctgcatcatcgaaattgccgtcaaccaagctctgatagagttggtcaagaccaatgcggagcatatacgcccggagtcgtggcgatcctgcaagctccggatgcctccgctcgaagtagcgcgtctgctgctccatacaagccaaccacggcctccagaagaagatgttggcgacctcgtattgggaatccccgaacattgcctcgctccagtcaatgaccgctgttatgcggccattgtccgtcaggacattgttggagccgaaatccgcgtgcacgaggtgccggacttcggggcagtcctcggcccaaagcatcagctcatcgagagcctgcgcgacggacgcactgacggtgtcgtccatcacagtttgccagtgatacacatggggatcagcaatcgcgcatatgaaatcacgccatgtagtgtattgaccgattccttgcggtccgaatgggccgaacccgctcgtctggctaagatcggccgcagcgatcgcatccatggcctccgcgaccggctgcagaacagcgggcagttcggtttcaggcaggtcttgcaacgtgacaccctgtgcacggcgggagatgcaataggtcaggctctcgctgaattccccaatgtcaagcacttccggaatcgggagcgcggccgatgcaaagtgccgataaacataacgatctttgtagaaaccatcggcgcagctatttacccgcaggacatatccacgccctcctacatcgaagctgaaagcacgagattcttcgccctccgagagctgcatcaggtcggacacgctgtcgaacttttcgatcagaaacttctcgacagacgtcgcggtgagttcaggctttttcattgcctcgatcgagttgagagtgaatatgagactctaattggataccgaggggaatttatggaacgtcagtggagcatttttgacaagaaatatttgctagctgatagtgaccttaggcgacttttgaacgcgcaataatggtttctgacgtatgtgcttagctcattaaactccagaaacccgcggctcagtggctccttcaacgttgcggttctgtcagttccaaacgtaaaacggcttgtcccgcgtcatcggcgggggtcataccgtgactcccttaattctcatgtatctccgtcaggagtccctaatgatattgttcacgtaattaagttttgtggaagtgagagagtccaattttgataagaaaagagtcagaaaacgtaatattttaaaagtctaaatctttctacaaataagagcaaatttatttattttttaatccaataaatattaatggaggacaaattcaattcacttggttgtaaaataaacttaaaccaataaccaaagaactaataaatcctgaagtggaattattaaggataaatgtacatagacaatgaagaaataataggttcgatgaattaataataattaaggatgttacaatcatcatgtgccaagtatatacacaatattctatgggatttataatttcgttacttcacttaacttttgcgtaaataaaacgaattatctgatattttataataaaacagttataagaaccatcatttttaacaacatagatatattatttctaatagtttaatgatacttttaaatcttttaaattttatgtttcttttagaaaataaaaattcaaaaaattaaatatatttacaaaaactacaatcaaacacaacttcatatattaaaagcaaaatatattttgaaaatttcaagtgtcctaacaaataagacaagaggaaaatgtacgatgagagacataaagagaactaataattgaggagtcctataatatataataaagtttattagtaaacttaattattaaggactcctaaaatatatgataggagaaaatgaatggtgagagatattggaaaacttaataattaaggattttaaaatatatggtaaaagataggcaaagtatccattatccccttttaacttgaagtctactaggcgcatgtgaaagttgattttttgtcacgtcatatagctataacgtaaaaaaagaaagtaaaatttttaattttttttaatatatgacatattttaaacgaaatataggacaaaatgtaaatgaatagtaaaggaaacaaagattaatacttactttgtaagaatttaagataaatttaaaatttaatagatcaactttacgtctagaaagacccatatctagaaggaatttcacgaaatcggcccttattcgaaaataacttttaaataatgaattttaaattttaagaaataatatccaatgaataaatgacatgtagcattttacctaaatatttcaactattttaatccaatattaatttgttttattcccaacaatagaaagtcttgtgcagacatttaatctgacttttccagtactaaatattaattttctgaagattttcgggtttagtccacaagttttagtgagaagttttgctcaaattttaggtgagaaggtttgatatttatcttttgttaaattaatttatctaggtgactattatttatttaagtagaaattcatatcattacttttgccaacttgtagtcataataggagtaggtgtatatgatgaaggaataaacaagttcagtgaagtgattaaaataaaatataatttaggtgtacatcaaataaaaaccttaaagtttagaaaggcaccgaataattttgcatagaagatattagtaaatttataaaaataaaagaaatgtagttgtcaagttgtcttcttttttttggataaaaatagcagttggcttatgtcattcttttacaacctccatgccacttgtccaattgttgacacttaactaattagtttgattcatgtatgaatactaaataattttttaggactgactcaaatatttttatattatcatagtaatatttatctaatttttaggaccacttattactaaataataaattaactacaactatattattgttgtgaaacaacaacgttttggttgttatgatgaaacgtacactatatcagtatgaaaaattcaaaacgattagtataaattatattgaaaatttgatatttttctattcttaatcagacgtattgggtttcatattttaaaaagggactaaacttagaagagaagtttgtttgaaactacttttgtctctttcttgttcccatttctctcttagatttcaaaaagtgaactactttatctccttctttgttcacattttattttattctattataaatatggcatcctcatattgagatttttagaaattattctaatcattcacagtgcaaaagaagaatggaatctcctgctactaaattacctgcacctctgctgatgttatcttcttctccattccttctcccttctcctaataagagctcctccatcttccttccacgtaaattagggccgctacctccaaaatattattattacaattgctgccatcctaagagtagatcaatctcagtagtatcaatggcaaataaggaggaggcagagacaagtaagaagaagcccaaaccattaaaagtactaattaccaaagtggatccgaagccgaggaagggcatggcatccgtcgcagtggacttactcgagaaggcctttgtatacctattgtccggaaattctgcagctgatcgtagtagtagtagtggtcgtcgtcgtcgtaaagagcattactacctctccggcaattatgcgcccgtcggacacgaaaccccgccctccgaccacctccccattcatggatcccttcctgaatgcttgaatggagtgtttctgagagttggtcctaaccccaagtttgctcccgtagccggatacaattgggtcgatggagatggaatgattcatggattgcgtattaaagatggaaaagcaacttatctatctcgatatattaaaacgtcacggtttaaacaagaagaatattttggaagagcaaaatttatgaagattggagatctaaggggattgcttgggttctttacgatcttaatactagtacttcgaacaacattgaaagtaatagacatttcatatggaagagggacgggtaatacagctcttgtgtatcataatggcttactattggctctatcagaagaagataaaccttatgttgttaaagttttagaagatggagacttgcaaactcttgggatattggattatgacaagaaattgtcacatccattcaccgctcatccaaagatcgatccgttaactgatgagatgtttacctttggatattccatctcgcctccgtatcttacttatcgagtcatttccaaggatggagtgatgcaagatccagtgcaaatctcaattacatcccctaccataatgcatgattttgctattactgaaaattatgccatcttcatggacctgcccttgtatttccaaccagaggaaatggtaaaggggaaatttgtctcttcatttcaccctacaaaaagagctcgtatcggtgtgcttccacgatatgcaaaagacgagcatccaattcgatggttcgatcttccaagttgcttcatgactcataatgcaaatgcttgggaagagaatgatgaagttgtgctattcacatgtcgccttgagagtcctgatcttgacatgcttagtggacctgcggaagaagagattgggaattcaaaaagtgagctttacgaaatgaggttcaatttgaaaactggaattacttcacaaaagcaactatctgtacctagtgttgattttcctcggatcaaccaaagttatactggcaggaaacagcaatatgtttattgtactcttggcaacaccaagattaagggcattgtgaagtttgatctgcaaattgaaccagaagccggaaagacaatgcttgaagttggaggaaatgtacaaggcatctttgagttgggacctagaagatatggttcagaggcaatatttgtgccatgccaacctggcatcaaatctgatgaggatgacggttacttgatattctttgtacacgacgaaaacaatgggaaatctgaggtcaatgtcatcgatgcaaagacaatgtctgcagaacctgtggctgttgtggaacttccaagcagggttccatatggattccatgccttgtttctgaatgaggaagaacttcagaagcaccaagcagagacatgagcttcggccatgctagagtccgcaaaaatcaccagtctctctctacaaatctatctctctctatttttctccagaataatgtgtgagtagttcccagataagggaattagggttcttatagggtttcgctcatgtgttgagcatataagaaacccttagtatgtatttgtatttgtaaaatacttctatcaataaaatttctaattcctaaaaccaaaatccagtgacctcgctgtcatgagacgaattctgacaggatatattggcgggtaaacctaagagaaaagagcgtttattagaataatcggatatttaaaagggcgtgaaaaggtttatccgttcgtccatttgtatgtgcatgccaaccacagggttcccctcgggatcaaagtactttgatccaacccctccgctgctatagtgcagtcggcttctgacgttcagtgcagccgtcatctgaaaacgacatgtcgcacaagtcctaagttacgcgacaggctgccgccctgcccttttcctggcgttttcttgtcgcgtgttttagtcgcataaagtagaatacttgcgactagaaccggagacattacgccatgaacaagagcgccgccgctggcctgctgggctatgcccgcgtcagcaccgacgaccaggacttgaccaaccaacgggccgaactgcacgcggccggctgcaccaagctgttttccgagaagatcaccggcaccaggcgcgaccgcccggagctggccaggatgcttgaccacctacgccctggcgacgttgtgacagtgaccaggctagaccgcctggcccgcagcacccgcgacctactggacattgccgagcgcatccaggaggccggcgcgggcctgcgtagcctggcagagccgtgggccgacaccaccacgccggccggccgcatggtgttgaccgtgttcgccggcattgccgagttcgagcgttccctaatcatcgaccgcacccggagcgggcgcgaggccgccaaggcccgaggcgtgaagtttggcccccgccctaccctcaccccggcacagatcgcgcacgcccgcgagctgatcgaccaggaaggccgcaccgtgaaagaggcggctgcactgcttggcgtgcatcgctcgaccctgtaccgcgcacttgagcgcagcgaggaagtgacgcccaccgaggccaggcggcgcggtgccttccgtgaggacgcattgaccgaggccgacgccctggcggccgccgagaatgaacgccaagaggaacaagcatgaaaccgcaccaggacggccaggacgaaccgtttttcattaccgaagagatcgaggcggagatgatcgcggccgggtacgtgttcgagccgcccgcgcacctctcaaccgtgcggctgcatgaaatcctggccggtttgtctgatgccaagctggcggcctggccggccagcttggccgctgaagaaaccgagcgccgccgtctaaaaaggtgatgtgtatttgagtaaaacagcttgcgtcatgcggtcgctgcgtatatgatccgatgagtaaataaacaaatacgcaaggggaacgcatgaaggttatcgctgtacttaaccagaaaggcgggtcaggcaagacgaccatcggaacccatctagcccgcgccctgcaactcgccggggccgatgttctgttagtcgattccgatccccagggcagtgcccgcgattgggcggccgtgcgggaagatcaaccgctaaccgttgtcggcatcgaccgcccgacgattgaccgcgacgtgaaggccatcggccggcgcgacttcgtagtgatcgacggagcgccccaggcggcggacttggctgtgtccgcgatcaaggcagccgacttcgtgctgattccggtgcagccaagcccttacgacatatgggccaccgccgacctggtggagctggttaagcagcgcattgaggtcacggatggaaggctacaagcggcctttgtcgtgtcgcgggcgatcaaaggcacgcgcatcggcggtgaggttgccgaggcgctggccgggtacgagctgcccattcttgagtcccgtatcacgcagcgcgtgagctacccaggcactgccgccgccggcacaaccgttcttgaatcagaacccgagggcgacgctgcccgcgaggtccaggcgctggccgctgaaattaaatcaaaactcatttgagttaatgaggtaaagagaaaatgagcaaaagcacaaacacgctaagtgccggccgtccgagcgcacgcagcagcaaggctgcaacgttggccagcctggcagacacgccagccatgaagcgggtcaactttcagttgccggcggaggatcacaccaagctgaagatgtacgcggtacgccaaggcaagaccattaccgagctgctatctgaatagatcgcgcagctaccagagtaaatgagcaaatgaataaatgagtagatgaattttagcggctaaaggaggcggcatggaaaatcaagaacaaccaggcaccgacgccgtggaatgccccatgtgtggaggaacgggcggttggccaggcgtaagcggctgggttgtctgccggccctgcaatggcactggaacccccaagcccgaggaatcggcgtgacggtcgcaaaccatccggcccggtacaaatcggcgcggcgctgggtgatgacctggtggagaagttgaaggccgcgcaggccgcccagcggcaacgcatcgaggcagaagcacgccccggtgaatcgtggcaagcggccgctgatcgaatccgcaaagaatcccggcaaccgccggcagccggtgcgccgtcgattaggaagccgcccaagggcgacgagcaaccagattttttcgttccgatgctctatgacgtgggcacccgcgatagtcgcagcatcatggacgtggccgttttccgtctgtcgaagcgtgaccgacgagctggcgaggtgatccgctacgagcttccagacgggcacgtagaggtttccgcagggccggccggcatggccagtgtgtgggattacgacctggtactgatggcggtttcccatctaaccgaatccatgaaccgataccgggaagggaagggagacaagcccggccgcgtgttccgtccacacgttgcggacgtactcaagttctgccggcgagccgatggcggaaagcagaaagacgacctggtagaaacctgcattcggttaaacaccacgcacgttgccatgcagcgtacgaagaaggccaagaacggccgcctggtgacggtatccgagggtgaagccttgattagccgctacaagatcgtaaagagcgaaaccgggcggccggagtacatcgagatcgagctagctgattggatgtaccgcgagatcacagaaggcaagaacccggacgtgctgacggttcaccccgattactttttgatcgatcccggcatcggccgttttctctaccgcctggcacgccgcgccgcaggcaaggcagaagccagatggttgttcaagacgatctacgaacgcagtggcagcgccggagagttcaagaagttctgtttcaccgtgcgcaagctgatcgggtcaaatgacctgccggagtacgatttgaaggaggaggcggggcaggctggcccgatcctagtcatgcgctaccgcaacctgatcgagggcgaagcatccgccggttcctaatgtacggagcagatgctagggcaaattgccctagcaggggaaaaaggtcgaaaaggactctttcctgtggatagcacgtacattgggaacccaaagccgtacattgggaaccggaacccgtacattgggaacccaaagccgtacattgggaaccggtcacacatgtaagtgactgatataaaagagaaaaaaggcgatttttccgcctaaaactctttaaaacttattaaaactcttaaaacccgcctggcctgtgcataactgtctggccagcgcacagccgaagagctgcaaaaagcgcctacccttcggtcgctgcgctccctacgccccgccgcttcgcgtcggcctatcgcggccgctggccgctcaaaaatggctggcctacggccaggcaatctaccagggcgcggacaagccgcgccgtcgccactcgaccgccggcgcccacatcaaggcaccctgcctcgcgcgtttcggtgatgacggtgaaaacctctgacacatgcagctcccggtgacggtcacagcttgtctgtaagcggatgccgggagcagacaagcccgtcagggcgcgtcagcgggtgttggcgggtgtcggggcgcagccatgacccagtcacgtagcgatagcggagtgtatactggcttaactatgcggcatcagagcagattgtactgagagtgcaccatatgcggtgtgaaataccgcacagatgcgtaaggagaaaataccgcatcaggcgctcttccgcttcctcgctcactgactcgctgcgctcggtcgttcggctgcggcgagcggtatcagctcactcaaaggcggtaatacggttatccacagaatcaggggataacgcaggaaagaacatgtgagcaaaaggccagcaaaaggccaggaaccgtaaaaaggccgcgttgctggcgtttttccataggctccgcccccctgacgagcatcacaaaaatcgacgctcaagtcagaggtggcgaaacccgacaggactataaagataccaggcgtttccccctggaagctccctcgtgcgctctcctgttccgaccctgccgcttaccggatacctgtccgcctttctcccttcgggaagcgtggcgctttctcatagctcacgctgtaggtatctcagttcggtgtaggtcgttcgctccaagctgggctgtgtgcacgaaccccccgttcagcccgaccgctgcgccttatccggtaactatcgtcttgagtccaacccggtaagacacgacttatcgccactggcagcagccactggtaacaggattagcagagcgaggtatgtaggcggtgctacagagttcttgaagtggtggcctaactacggctacactagaaggacagtatttggtatctgcgctctgctgaagccagttaccttcggaaaaagagttggtagctcttgatccggcaaacaaaccaccgctggtagcggtggtttttttgtttgcaagcagcagattacgcgcagaaaaaaaggatctcaagaagatcctttgatcttttctacggggtctgacgctcagtggaacgaaaactcacgttaagggattttggtcatgcattctaggtgattagaaaaactcatcgagcatcaaatgaaactgcaatttattcatatcaggattatcaataccatatttttgaaaaagccgtttctgtaatgaaggagaaaactcaccgaggcagttccataggatggcaagatcctggtatcggtctgcgattccgactcgtccaacatcaatacaacctattaatttcccctcgtcaaaaataaggttatcaagtgagaaatcaccatgagtgacgactgaatccggtgagaatggcaaaagtttatgcatttctttccagacttgttcaacaggccagccattacgctcgtcatcaaaatcactcgcatcaaccaaaccgttattcattcgtgattgcgcctgagcgagtcgaaatacgcgatcgctgttaaaaggacaattacaaacaggaatcgaatgcaaccggcgcaggaacactgccagcgcatcaacaatattttcacctgaatcaggatattcttctaatacctggaatgctgttttccctgggatcgcagtggtgagtaaccatgcatcatcaggagtacggataaaatgcttgatggtcggaagaggcataaattccgtcagccagtttagtctgaccatctcatctgtaacatcattggcaacgctacctttgccatgtttcagaaacaactctggcgcatcgggcttcccatacaatcggtagattgtcgcacctgattgcccgacattatcgcgagcccatttatacccatataaatcagcatccatgttggaatttaatcgcggccttgagcaagacgtttcccgttgaatatggctcataacagaacttattatttccttcctcttttctacagtatttaaagataccccaagaagctaattataacaagacgaactccaattcactgttccttgcattctaaaaccttaaataccagaaaacagctttttcaaagttgttttcaaagttggcgtataacatagtatcgacggagccgattttgaaaccgcggtgatcacaggcagcaacgctctgtcatcgttacaatcaacatgctaccctccgcgagatcatccgtgtttcaaacccggcagcttagttgccgttcttccgaatagcatcggtaacatgagcaaagtctgccgccttacaacggctctcccgctgacgccgtcccggactgatgggctgcctgtatcgagtggtgattttgtgccgagctgccggtcggggagctgttggctggctggtggcaggatatattgtggtgtaaacataacgaattcgtctca

SEQ ID NO: 23 - DNA, 16761 bp, Artificial Sequence
  DNA contruct O3 = = pDGB3?1[p35S:UGT2:T35S-p35S:UGT709G1:T35S-p35S:CCD2L:T35S-pNos:Hy g:T35S]
ggagactagagccaagctgatctcctttgccccggagatcaccatggacgactttctctatctctacgatctaggaagaaagttcgacggagaaggtgacgataccatgttcaccaccgataatgagaagattagcctcttcaatttcagaaagaatgctgacccacagatggttagagaggcctacgcggcaggtctgatcaagacgatctacccgagtaataatctccaggagatcaaataccttcccaagaaggttaaagatgcagtcaaaagattcaggactaactgcatcaagaacacagagaaagatatatttctcaagatcagaagtactattccagtatggacgattcaaggcttgcttcataaaccaaggcaagtaatagagattggagtctctaagaaagtagttcctactgaatcaaaggccatggagtcaaaaattcagatcgaggatctaacagaactcgccgtgaagactggcgaacagttcatacagagtcttttacgactcaatgacaagaagaaaatcttcgtcaacatggtggagcacgacactctcgtctactccaagaatatcaaagatacagtctcagaagaccaaagggctattgagacttttcaacaaagggtaatatcgggaaacctcctcggattccattgcccagctatctgtcacttcatcaaaaggacagtagaaaaggaaggtggcacctacaaatgccatcattgcgataaaggaaaggctatcgttcaagatgcctctgccgacagtggtcccaaagatggacccccacccacgaggagcatcgtggaaaaagaagacgttccaaccacgtcttcaaagcaagtggattgatgtgatatctccactgacgtaagggatgacgcacaatcccactatccttcgcaagacccttcctctatataaggaagttcatttcatttggagaggactccggtatttttacaacaataccacaacaaaacaaacaacaaacaacattacaatttactattctagtcgaaatgttgaacggcaacaaatgccacatcctcctcctcccctgtccagcacaaggccatatcaaccccattctccaattcggcaagcgactggcctctcacaacctcctcaccacactcgtcaacacccggttcctctccaactcgaccaaatccgaacccggtccggtcaacatccagtgcatatccgacggattcgatcccggtgggatgaatgcagcacctagtcgtcgggcctatttcgaccgacctcagagtcggtcgggtcagaaacatgttggcctcatcgagtcactccggtccagaggccgacccggcgcatgttttggtctacgacccgttcccctctgggcaatgaacgtagccgagcggtccgggctgcggtcggtcgcattctttactcagccgtgtgcagtggacacaatctaccgccacgtgtgggagggacgaattaaggttccggttgccgagccggtccggttgcctggattgcccccactcgagcctagtgatctgccgtgcgttcgtaacggattcggacgagtcgttaacccggatctcttgccacttcgagtgaatcagcacaaaaatttggacaaagctgacatgatggggaggaactccatatacgagctagaggcggatttgttggatgggtcccgattaccattaccggtgaagtcgattgggccgaccgtgccgtctacttatctcgacaaccgaatcccgtcggattcacactatggattcaatctatacacccctgacactactccctacttggactggctcgactccaaggccccgaactctgtcatctatgtctcatttggtagtttgtccagtctgagccctgatcaaaccaatgagattgcgtcgggtctgatcgccaccaacaaaagctttatttgggtggtacgcacttcggagttagccaaactccctgccaacttcacccaagagaatgcgagccgtgggctggttgtgacctggtgcgaccaactcgatctcctcgcacacgttgcgaccggttgcttcgtgactcactgcggatggaactcgactatggaaggtgtcgcacttggtgtgccgatggtgggagtgccgcagtggtcggaccagcctatgaatgccaagtatgtagaggatgtgtggaaggtcggcgtgagggcgaagacttatgggaaggattttgtgagaggggaggagttcaaaagatgtgtggaggaggtgatggatggagagaggagtggaaagattagagagaatgccgcaaggtggtgtaagttggccaaggactctgttagtgagggtgggagttctgacaagtgtatcaaggagttcatacatcagtgttgcaatgactccaaaatttccttagtttaagcttcggccatgctagagtccgcaaaaatcaccagtctctctctacaaatctatctctctctatttttctccagaataatgtgtgagtagttcccagataagggaattagggttcttatagggtttcgctcatgtgttgagcatataagaaacccttagtatgtatttgtatttgtaaaatacttctatcaataaaatttctaattcctaaaaccaaaatccagtgacctcgctgtcaggagactagagccaagctgatctcctttgccccggagatcaccatggacgactttctctatctctacgatctaggaagaaagttcgacggagaaggtgacgataccatgttcaccaccgataatgagaagattagcctcttcaatttcagaaagaatgctgacccacagatggttagagaggcctacgcggcaggtctgatcaagacgatctacccgagtaataatctccaggagatcaaataccttcccaagaaggttaaagatgcagtcaaaagattcaggactaactgcatcaagaacacagagaaagatatatttctcaagatcagaagtactattccagtatggacgattcaaggcttgcttcataaaccaaggcaagtaatagagattggagtctctaagaaagtagttcctactgaatcaaaggccatggagtcaaaaattcagatcgaggatctaacagaactcgccgtgaagactggcgaacagttcatacagagtcttttacgactcaatgacaagaagaaaatcttcgtcaacatggtggagcacgacactctcgtctactccaagaatatcaaagatacagtctcagaagaccaaagggctattgagacttttcaacaaagggtaatatcgggaaacctcctcggattccattgcccagctatctgtcacttcatcaaaaggacagtagaaaaggaaggtggcacctacaaatgccatcattgcgataaaggaaaggctatcgttcaagatgcctctgccgacagtggtcccaaagatggacccccacccacgaggagcatcgtggaaaaagaagacgttccaaccacgtcttcaaagcaagtggattgatgtgatatctccactgacgtaagggatgacgcacaatcccactatccttcgcaagacccttcctctatataaggaagttcatttcatttggagaggactccggtatttttacaacaataccacaacaaaacaaacaacaaacaacattacaatttactattctagtcgaaatggctgagaaagaagcaaatacccatgtcgtcctcttccccttgccaggccaagggcacatcggctcaatgttgaaactggcacagcttctttccaccgccggattctacgtcactttcgtccacaccgaacgcaactaccgtcgctacctcctcacctccacgtccttccacgtccccaagttccggttccgcaccatccccgacggttttcccgacgacgattcccgctcgcccctcccttttctcgagctccaagagtcgctggacacgaaatgtcgggggcattatcgggaattgttggtcgctgtcgacgaccaagaagagtggcccccagtcacttgtgtcgtggctgatcaagctcttccactctcactcgaagttcccgacgagttggggattcctgtaatgatactcgcaccacacagtgcgtgcagtatattgacgagttattcgattccggagcttataaggggaggtgaactccctatcccagatggggccaatatggatgaactattacaaggcgtactgggattggaaggtatcgtgaggcgtagggatatgtccatcagaagcgccaagtccatccaagatccatttcttcaattcgaagtgaaaatgagcaaaaacttgcccagaggaagagctctcatcctgaacactacagaatcgatagactctctttctttgcgacacattcggtcgatctgtcccactacctacgcactcgggcccttccacgtccttctcaggaacataaaagacgagtcccactccgcaagcctttccgaagaggacaggtcctgcatcgcctggctggactcgaaaccgaacaagtccgcggtctacgtgagtttcggtagcctcgccgccatggcgagagaagcatttcttgagtttcagcagggattgctcgacagcgggtattacttcttgtgggtgatccggcccgatatggtggaaggggggctggaagagagcgagctgaccgcgagcgaacaacgctactttgtgaagtgggccccacaggaggaggttcttgcgcacccggcggtagggtgtttcttgacgcacagcggttggaactctacgttggagagtatctttgcgggagtgccgatgatatgttggcctttctttgcggaccagctgattaacagtaggtttgcgagcgaggtgtggaaaattgccttggatatgaaggatttgtgcggaaggagccacgtggagaggatggtgaaggaagttatgagtggagagaaaggcgaagagctaaggaattctagctgcgagatggcagatagggtgaagaagagtgcagaggaaggtggctcttcctacgccaacttcaaagagttggttggacatatcaaatctttgagcttaccagcagaaagaggagaaaatggtggtgaaggaatgagtgtacaagcgccgagtaaacttttcctcctcaacgctgaggacggaaaacatgtccttaaaagtgacgaaccgtcggaacaaaggggtccacaatttaatccaaattttcttcggacctgagcttcggccatgctagagtccgcaaaaatcaccagtctctctctacaaatctatctctctctatttttctccagaataatgtgtgagtagttcccagataagggaattagggttcttatagggtttcgctcatgtgttgagcatataagaaacccttagtatgtatttgtatttgtaaaatacttctatcaataaaatttctaattcctaaaaccaaaatccagtgacctcgctgtcaggagagcgcgagtcggtcccattattgaagcatttatcagggttattgtctcatgagcggatacatatttgaatgtatttagaaaaataaacaaataggggttccgcgcacatttccccgaaaagtgccacctgacgtctaagaaaccattattatcatgacattaacctataaaaataggcgtatcacgaggccctttcgtcttcaagaattagcttggcaattcccgatctagtaacatagatgacaccghgcgcgataatttatcctagtttgcgcgctatattttgttttctatcgcgtattaaatgtataattgcgggactctaatcataaaaacccatctcataaataacgtcatgcattacatgttaattattacatgcttaacgtaattcaacagaaattatatgataatcgtcgcaagaccggcaacaggattcaatcttaagaaactttattgccaaatgtttgaacgatcgggatcgaagatccattccaagctcattcctttgccctcggacgagtgctggggcgtcggtttccactatcggcgagtacttctacacagccatcggtccagacggccgcgcttctgcgggcgatttgtgtacgcccgacagtcccggctccggatcggacgattgcgtcgcatcgaccctgcgcccaagctgcatcatcgaaattgccgtcaaccaagctctgatagagttggtcaagaccaatgcggagcatatacgcccggagtcgtggcgatcctgcaagctccggatgcctccgctcgaagtagcgcgtctgctgctccatacaagccaaccacggcctccagaagaagatgttggcgacctcgtattgggaatccccgaacattgcctcgctccagtcaatgaccgctgttatgcggccattgtccgtcaggacattgttggagccgaaatccgcgtgcacgaggtgccggacttcggggcagtcctcggcccaaagcatcagctcatcgagagcctgcgcgacggacgcactgacggtgtcgtccatcacagtttgccagtgatacacatggggatcagcaatcgcgcatatgaaatcacgccatgtagtgtattgaccgattccttgcggtccgaatgggccgaacccgctcgtctggctaagatcggccgcagcgatcgcatccatggcctccgcgaccggctgcagaacagcgggcagttcggtttcaggcaggtcttgcaacgtgacaccctgtgcacggcgggagatgcaataggtcaggctctcgctgaattccccaatgtcaagcacttccggaatcgggagcgcggccgatgcaaagtgccgataaacataacgatctttgtagaaaccatcggcgcagctatttacccgcaggacatatccacgccctcctacatcgaagctgaaagcacgagattcttcgccctccgagagctgcatcaggtcggacacgctgtcgaacttttcgatcagaaacttctcgacagacgtcgcggtgagttcaggctttttcattgcctcgatcgagttgagagtgaatatgagactctaattggataccgaggggaatttatggaacgtcagtggagcatttttgacaagaaatatttgctagctgatagtgaccttaggcgacttttgaacgcgcaataatggtttctgacgtatgtgcttagctcattaaactccagaaacccgcggctcagtggctccttcaacgttgcggttctgtcagttccaaacgtaaaacggcttgtcccgcgtcatcggcgggggtcataccgtgactcccttaattctcatgtatctccgtcaggagactagagccaagctgatctcctttgccccggagatcaccatggacgactttctctatctctacgatctaggaagaaagttcgacggagaaggtgacgataccatgttcaccaccgataatgagaagattagcctcttcaatttcagaaagaatgctgacccacagatggttagagaggcctacgcggcaggtctgatcaagacgatctacccgagtaataatctccaggagatcaaataccttcccaagaaggttaaagatgcagtcaaaagattcaggactaactgcatcaagaacacagagaaagatatatttctcaagatcagaagtactattccagtatggacgattcaaggcttgcttcataaaccaaggcaagtaatagagattggagtctctaagaaagtagttcctactgaatcaaaggccatggagtcaaaaattcagatcgaggatctaacagaactcgccgtgaagactggcgaacagttcatacagagtcttttacgactcaatgacaagaagaaaatcttcgtcaacatggtggagcacgacactctcgtctactccaagaatatcaaagatacagtctcagaagaccaaagggctattgagacttttcaacaaagggtaatatcgggaaacctcctcggattccattgcccagctatctgtcacttcatcaaaaggacagtagaaaaggaaggtggcacctacaaatgccatcattgcgataaaggaaaggctatcgttcaagatgcctctgccgacagtggtcccaaagatggacccccacccacgaggagcatcgtggaaaaagaagacgttccaaccacgtcttcaaagcaagtggattgatgtgatatctccactgacgtaagggatgacgcacaatcccactatccttcgcaagacccttcctctatataaggaagttcatttcatttggagaggactccggtatttttacaacaataccacaacaaaacaaacaacaaacaacattacaatttactattctagtcgaaatgcatggaatctcctactactaaattacctgcacctctgctgatgttatcttcttctccactccttctcccttctccttataagagctcctccatcttccttccacgtaaatttgggccgctacctcctaattattattacaattgctgccatcctaagagtagaccaatctcagtagtatcaatggcaaataaggaggaggcagagaagaggaagaagaagcccaaaccattaaaagtactaattaccaaagtggacccgaagccgaggaagggcatggcatccgtcgcagtggacttactcgagaaggcctttgtatacctattgtacggaaattctgcagctgatcgtagtagtggtcgtcgtcgtcgtaaagagcattactacctctccggcaattatgcgcccgtcggacacgaaaccccaccctccgaccacctccccgttcatggatcccttcctgaatgcttgaatggagtgtttctgagagttggccctaaccccaagtttgctcccgtagccggatacaattgggtcgatggagatggaatgattcatggattgcgtattaaagatggaaaagcaacttatctatcccgatatattaaaacgtcacggtttaaacaagaagaatattttggaagagcaaaatttatgaagattggagatctaagaggattgcttggattctttacgatcttaatactagtacttcgaacaacattgaaagtaatagacatttcatatggaagggggacaggtaatacagctcttgtatatcataatggcttactattggctctatcagaagaagataaaccttatgttgttaaagttttagaagatggagacttgcaaactcttgggatattggattatgacaagaaattgtcacatccattcaccgctcatccaaagatcgatccgttaaccgatgagatgtttacctttggatattccctctcgcctccgtatcttacttatcgagtcatttccaaggatggagtgatgcaagatccagtgcaaatctcaattacatcccctaccataatgcatgattttgctattactgaaaattatgccatcttcatggacctgcccttgtatttccaaccagaggaaatggtaaaggggaaatttgtctcttcatttcaccccacaaaaagagctcgtatcggtgtgcttccacgatatgcagaagacgagcatccaattcgatggtttgatcttccaagttgcttcatgactcataatgcaaatgcttgggaagagaatgatgaagttgtgctattcacatgtcgccttgagagtcctgatcttgacatgcttagtggacctgcggaagaagagattgggaattcaaaaagtgagctttatgaaatgaggttcaatttgaaaactggaattacttcacaaaagcaactatctgtacctagtgttgattttcctcggatcaaccaaagttatactggcaggaaacagcaatatgtttattgtactcttggcaacaccaagattaagggcattgtgaagtttgatctgcaaattgaaccagaagccggaaagacaatgcttgaagttggaggaaatgtacaaggcatctttgagttgggacctagaagatatggttcagaggcaatatttgtgccatgccaacctggcatcaaatctgatgaggatgacggttacttgatattctttgtacacgacgaaaacaatgggaaatctgaggtcaatgtcatcgatgcaaagacaatgtctgcagaacctgtggctgttgtgcaacttccaagcagggttccatatggattccatgccttgtttgagcttcggccatgctagagtccgcaaaaatcaccagtctctctctacaaatctatctctctctatttttctccagaataatgtgtgagtagttcccagataagggaattagggttcttatagggtttcgctcatgtgttgagcatataagaaacccttagtatgtatttgtatttgtaaaatacttctatcaataaaatttctaattcctaaaaccaaaatccagtgacctcgctgtcatgagacgaattctgacaggatatattggcgggtaaacctaagagaaaagagcgtttattagaataatcggatatttaaaagggcgtgaaaaggtttatccgttcgtccatttgtatgtgcatgccaaccacagggttcccctcgggatcaaagtactttgatccaacccctccgctgctatagtgcagtcggcttctgacgttcagtgcagccgtcatctgaaaacgacatgtcgcacaagtcctaagttacgcgacaggctgccgccctgcccttttcctggcgttttcttgtcgcgtgttttagtcgcataaagtagaatacttgcgactagaaccggagacattacgccatgaacaagagcgccgccgctggcctgctgggctatgcccgcgtcagcaccgacgaccaggacttgaccaaccaacgggccgaactgcacgcggccggctgcaccaagctgttttccgagaagatcaccggcaccaggcgcgaccgcccggagctggccaggatgcttgaccacctacgccctggcgacgttgtgacagtgaccaggctagaccgcctggcccgcagcacccgcgacctactggacattgccgagcgcatccaggaggccggcgcgggcctgcgtagcctggcagagccgtgggccgacaccaccacgccggccggccgcatggtgttgaccgtgttcgccggcattgccgagttcgagcgttccctaatcatcgaccgcacccggagcgggcgcgaggccgccaaggcccgaggcgtgaagtttggcccccgccctaccctcaccccggcacagatcgcgcacgcccgcgagctgatcgaccaggaaggccgcaccgtgaaagaggcggctgcactgcttggcgtgcatcgctcgaccctgtaccgcgcacttgagcgcagcgaggaagtgacgcccaccgaggccaggcggcgcggtgccttccgtgaggacgcattgaccgaggccgacgccctggcggccgccgagaatgaacgccaagaggaacaagcatgaaaccgcaccaggacggccaggacgaaccgtttttcattaccgaagagatcgaggcggagatgatcgcggccgggtacgtgttcgagccgcccgcgcacctctcaaccgtgcggctgcatgaaatcctggccggtttgtctgatgccaagctggcggcctggccggccagcttggccgctgaagaaaccgagcgccgccgtctaaaaaggtgatgtgtatttgagtaaaacagcttgcgtcatgcggtcgctgcgtatatgatccgatgagtaaataaacaaatacgcaaggggaacgcatgaaggttatcgctgtacttaaccagaaaggcgggtcaggcaagacgaccatcggaacccatctagcccgcgccctgcaactcgccggggccgatgttctgttagtcgattccgatccccagggcagtgcccgcgattgggcggccgtgcgggaagatcaaccgctaaccgttgtcggcatcgaccgcccgacgattgaccgcgacgtgaaggccatcggccggcgcgacttcgtagtgatcgacggagcgccccaggcggcggacttggctgtgtccgcgatcaaggcagccgacttcgtgctgattccggtgcagccaagcccttacgacatatgggccaccgccgacctggtggagctggttaagcagcgcattgaggtcacggatggaaggctacaagcggcctttgtcgtgtcgcgggcgatcaaaggcacgcgcatcggcggtgaggttgccgaggcgctggccgggtacgagctgcccattcttgagtcccgtatcacgcagcgcgtgagctacccaggcactgccgccgccggcacaaccgttcttgaatcagaacccgagggcgacgctgcccgcgaggtccaggcgctggccgctgaaattaaatcaaaactcatttgagttaatgaggtaaagagaaaatgagcaaaagcacaaacacgctaagtgccggccgtccgagcgcacgcagcagcaaggctgcaacgttggccagcctggcagacacgccagccatgaagcgggtcaactttcagttgccggcggaggatcacaccaagctgaagatgtacgcggtacgccaaggcaagaccattaccgagctgctatctgaatagatcgcgcagctaccagagtaaatgagcaaatgaataaatgagtagatgaattttagcggctaaaggaggcggcatggaaaatcaagaacaaccaggcaccgacgccgtggaatgccccatgtgtggaggaacgggcggttggccaggcgtaagcggctgggttgtctgccggccctgcaatggcactggaacccccaagcccgaggaatcggcgtgacggtcgcaaaccatccggcccggtacaaatcggcgcggcgctgggtgatgacctggtggagaagttgaaggccgcgcaggccgcccagcggcaacgcatcgaggcagaagcacgccccggtgaatcgtggcaagcggccgctgatcgaatccgcaaagaatcccggcaaccgccggcagccggtgcgccgtcgattaggaagccgcccaagggcgacgagcaaccagattttttcgttccgatgctctatgacgtgggcacccgcgatagtcgcagcatcatggacgtggccgttttccgtctgtcgaagcgtgaccgacgagctggcgaggtgatccgctacgagcttccagacgggcacgtagaggtttccgcagggccggccggcatggccagtgtgtgggattacgacctggtactgatggcggtttcccatctaaccgaatccatgaaccgataccgggaagggaagggagacaagcccggccgcgtgttccgtccacacgttgcggacgtactcaagttctgccggcgagccgatggcggaaagcagaaagacgacctggtagaaacctgcattcggttaaacaccacgcacgttgccatgcagcgtacgaagaaggccaagaacggccgcctggtgacggtatccgagggtgaagccttgattagccgctacaagatcgtaaagagcgaaaccgggcggccggagtacatcgagatcgagctagctgattggatgtaccgcgagatcacagaaggcaagaacccggacgtgctgacggttcaccccgattactttttgatcgatcccggcatcggccgttttctctaccgcctggcacgccgcgccgcaggcaaggcagaagccagatggttgttcaagacgatctacgaacgcagtggcagcgccggagagttcaagaagttctgtttcaccgtgcgcaagctgatcgggtcaaatgacctgccggagtacgatttgaaggaggaggcggggcaggctggcccgatcctagtcatgcgctaccgcaacctgatcgagggcgaagcatccgccggttcctaatgtacggagcagatgctagggcaaattgccctagcaggggaaaaaggtcgaaaaggactctttcctgtggatagcacgtacattgggaacccaaagccgtacattgggaaccggaacccgtacattgggaacccaaagccgtacattgggaaccggtcacacatgtaagtgactgatataaaagagaaaaaaggcgatttttccgcctaaaactctttaaaacttattaaaactcttaaaacccgcctggcctgtgcataactgtctggccagcgcacagccgaagagctgcaaaaagcgcctacccttcggtcgctgcgctccctacgccccgccgcttcgcgtcggcctatcgcggccgctggccgctcaaaaatggctggcctacggccaggcaatctaccagggcgcggacaagccgcgccgtcgccactcgaccgccggcgcccacatcaaggcaccctgcctcgcgcgtttcggtgatgacggtgaaaacctctgacacatgcagctcccggtgacggtcacagcttgtctgtaagcggatgccgggagcagacaagcccgtcagggcgcgtcagcgggtgttggcgggtgtcggggcgcagccatgacccagtcacgtagcgatagcggagtgtatactggcttaactatgcggcatcagagcagattgtactgagagtgcaccatatgcggtgtgaaataccgcacagatgcgtaaggagaaaataccgcatcaggcgctcttccgcttcctcgctcactgactcgctgcgctcggtcgttcggctgcggcgagcggtatcagctcactcaaaggcggtaatacggttatccacagaatcaggggataacgcaggaaagaacatgtgagcaaaaggccagcaaaaggccaggaaccgtaaaaaggccgcgttgctggcgtttttccataggctccgcccccctgacgagcatcacaaaaatcgacgctcaagtcagaggtggcgaaacccgacaggactataaagataccaggcgtttccccctggaagctccctcgtgcgctctcctgttccgaccctgccgcttaccggatacctgtccgcctttctcccttcgggaagcgtggcgctttctcatagctcacgctgtaggtatctcagttcggtgtaggtcgttcgctccaagctgggctgtgtgcacgaaccccccgttcagcccgaccgctgcgccttatccggtaactatcgtcttgagtccaacccggtaagacacgacttatcgccactggcagcagccactggtaacaggattagcagagcgaggtatgtaggcggtgctacagagttcttgaagtggtggcctaactacggctacactagaaggacagtatttggtatctgcgctctgctgaagccagttaccttcggaaaaagagttggtagctcttgatccggcaaacaaaccaccgctggtagcggtggtttttttgtttgcaagcagcagattacgcgcagaaaaaaaggatctcaagaagatcctttgatcttttctacggggtctgacgctcagtggaacgaaaactcacgttaagggattttggtcatgcattctaggtgattagaaaaactcatcgagcatcaaatgaaactgcaatttattcatatcaggattatcaataccatatttttgaaaaagccgtttctgtaatgaaggagaaaactcaccgaggcagttccataggatggcaagatcctggtatcggtctgcgattccgactcgtccaacatcaatacaacctattaatttcccctcgtcaaaaataaggttatcaagtgagaaatcaccatgagtgacgactgaatccggtgagaatggcaaaagtttatgcatttctttccagacttgttcaacaggccagccattacgctcgtcatcaaaatcactcgcatcaaccaaaccgttattcattcgtgattgcgcctgagcgagtcgaaatacgcgatcgctgttaaaaggacaattacaaacaggaatcgaatgcaaccggcgcaggaacactgccagcgcatcaacaatattttcacctgaatcaggatattcttctaatacctggaatgctgttttccctgggatcgcagtggtgagtaaccatgcatcatcaggagtacggataaaatgcttgatggtcggaagaggcataaattccgtcagccagtttagtctgaccatctcatctgtaacatcattggcaacgctacctttgccatgtttcagaaacaactctggcgcatcgggcttcccatacaatcggtagattgtcgcacctgattgcccgacattatcgcgagcccatttatacccatataaatcagcatccatgttggaatttaatcgcggccttgagcaagacgtttcccgttgaatatggctcataacagaacttattatttccttcctcttttctacagtatttaaagataccccaagaagctaattataacaagacgaactccaattcactgttccttgcattctaaaaccttaaataccagaaaacagctttttcaaagttgttttcaaagttggcgtataacatagtatcgacggagccgattttgaaaccgcggtgatcacaggcagcaacgctctgtcatcgttacaatcaacatgctaccctccgcgagatcatccgtgtttcaaacccggcagcttagttgccgttcttccgaatagcatcggtaacatgagcaaagtctgccgccttacaacggctctcccgctgacgccgtcccggactgatgggctgcctgtatcgagtggtgattttgtgccgagctgccggtcggggagctgttggctggctggtggcaggatatattgtggtgtaaacataacgaattcgtctca

SEQ ID NO: 24 - DNA, 20976 bp, Artificial Sequence
  DNA construct O4 = pDGB3?1[pE8:UGT2:T35S-p35S:UGT709G1:T35S-p2A11:CCD2L:T35S-pNos:Hy g:T35S]
ggagtccctaatgatattgttcacgtaattaagttttgtggaagtgagagagtccaattttgataagaaaagagtcagaaaacgtaatattttaaaagtctaaatctttctacaaataagagcaaatttatttattttttaatccaataaatattaatggaggacaaattcaattcacttggttgtaaaataaacttaaaccaataaccaaagaactaataaatcctgaagtggaattattaaggataaatgtacatagacaatgaagaaataataggttcgatgaattaataataattaaggatgttacaatcatcatgtgccaagtatatacacaatattctatgggatttataatttcgttacttcacttaacttttgcgtaaataaaacgaattatctgatattttataataaaacagttataagaaccatcatttttaacaacatagatatattatttctaatagtttaatgatacttttaaatcttttaaattttatgtttcttttagaaaataaaaattcaaaaaattaaatatatttacaaaaactacaatcaaacacaacttcatatattaaaagcaaaatatattttgaaaatttcaagtgtcctaacaaataagacaagaggaaaatgtacgatgagagacataaagagaactaataattgaggagtcctataatatataataaagtttattagtaaacttaattattaaggactcctaaaatatatgataggagaaaatgaatggtgagagatattggaaaacttaataattaaggattttaaaatatatggtaaaagataggcaaagtatccattatccccttttaacttgaagtctactaggcgcatgtgaaagttgattttttgtcacgtcatatagctataacgtaaaaaaagaaagtaaaatttttaattttttttaatatatgacatattttaaacgaaatataggacaaaatgtaaatgaatagtaaaggaaacaaagattaatacttactttgtaagaatttaagataaatttaaaatttaatagatcaactttacgtctagaaagacccatatctagaaggaatttcacgaaatcggcccttattcgaaaataacttttaaataatgaattttaaattttaagaaataatatccaatgaataaatgacatgtagcattttacctaaatatttcaactattttaatccaatattaatttgttttattcccaacaatagaaagtcttgtgcagacatttaatctgacttttccagtactaaatattaattttctgaagattttcgggtttagtccacaagttttagtgagaagttttgctcaaattttaggtgagaaggtttgatatttatcttttgttaaattaatttatctaggtgactattatttatttaagtagaaattcatatcattacttttgccaacttgtagtcataataggagtaggtgtatatgatgaaggaataaacaagttcagtgaagtgattaaaataaaatataatttaggtgtacatcaaataaaaaccttaaagtttagaaaggcaccgaataattttgcatagaagatattagtaaatttataaaaataaaagaaatgtagttgtcaagttgtcttcttttttttggataaaaatagcagttggcttatgtcattcttttacaacctccatgccacttgtccaattgttgacacttaactaattagtttgattcatgtatgaatactaaataattttttaggactgactcaaatatttttatattatcatagtaatatttatctaatttttaggaccacttattactaaataataaattaactacaactatattattgttgtgaaacaacaacgttttggttgttatgatgaaacgtacactatatcagtatgaaaaattcaaaacgattagtataaattatattgaaaatttgatatttttctattcttaatcagacgtattgggtttcatattttaaaaagggactaaacttagaagagaagtttgtttgaaactacttttgtctctttcttgttcccatttctctcttagatttcaaaaagtgaactactttatctccttctttgttcacattttattttattctattataaatatggcatcctcatattgagatttttagaaattattctaatcattcacagtgcaaaagaagaatgttgaacggcaacaaatgccacatcctcctcctcccctgtccagcacaaggccatatcaaccccattctccaattcggcaagcgactggcctctcacaacctcctcaccacactcgtcaacacccggttcctctccaactcgaccaaatccgaacccggtccggtcaacatccagtgcatatccgacggattcgatcccggtgggatgaatgcagcacctagtcgtcgggcctatttcgaccgacctcagagtcggtcgggtcagaaacatgttggcctcatcgagtcactccggtccagaggccgacccggcgcatgttttggtctacgacccgttcccctctgggcaatgaacgtagccgagcggtccgggctgcggtcggtcgcattctttactcagccgtgtgcagtggacacaatctaccgccacgtgtgggagggacgaattaaggttccggttgccgagccggtccggttgcctggattgcccccactcgagcctagtgatctgccgtgcgttcgtaacggattcggacgagtcgttaacccggatctcttgccacttcgagtgaatcagcacaaaaatttggacaaagctgacatgatggggaggaactccatatacgagctagaggcggatttgttggatgggtcccgattaccattaccggtgaagtcgattgggccgaccgtgccgtctacttatctcgacaaccgaatcccgtcggattcacactatggattcaatctatacacccctgacactactccctacttggactggctcgactccaaggccccgaactctgtcatctatgtctcatttggtagtttgtccagtctgagccctgatcaaaccaatgagattgcgtcgggtctgatcgccaccaacaaaagctttatttgggtggtacgcacttcggagttagccaaactccctgccaacttcacccaagagaatgcgagccgtgggctggttgtgacctggtgcgaccaactcgatctcctcgcacacgttgcgaccggttgcttcgtgactcactgcggatggaactcgactatggaaggtgtcgcacttggtgtgccgatggtgggagtgccgcagtggtcggaccagcctatgaatgccaagtatgtagaggatgtgtggaaggtcggcgtgagggcgaagacttatgggaaggattttgtgagaggggaggagttcaaaagatgtgtggaggaggtgatggatggagagaggagtggaaagattagagagaatgccgcaaggtggtgtaagttggccaaggactctgttagtgagggtgggagttctgacaagtgtatcaaggagttcatacatcagtgttgcaatgactccaaaatttccttagtttaagcttcggccatgctagagtccgcaaaaatcaccagtctctctctacaaatctatctctctctatttttctccagaataatgtgtgagtagttcccagataagggaattagggttcttatagggtttcgctcatgtgttgagcatataagaaacccttagtatgtatttgtatttgtaaaatacttctatcaataaaatttctaattcctaaaaccaaaatccagtgacctcgctgtcaggagactagagccaagctgatctcctttgccccggagatcaccatggacgactttctctatctctacgatctaggaagaaagttcgacggagaaggtgacgataccatgttcaccaccgataatgagaagattagcctcttcaatttcagaaagaatgctgacccacagatggttagagaggcctacgcggcaggtctgatcaagacgatctacccgagtaataatctccaggagatcaaataccttcccaagaaggttaaagatgcagtcaaaagattcaggactaactgcatcaagaacacagagaaagatatatttctcaagatcagaagtactattccagtatggacgattcaaggcttgcttcataaaccaaggcaagtaatagagattggagtctctaagaaagtagttcctactgaatcaaaggccatggagtcaaaaattcagatcgaggatctaacagaactcgccgtgaagactggcgaacagttcatacagagtcttttacgactcaatgacaagaagaaaatcttcgtcaacatggtggagcacgacactctcgtctactccaagaatatcaaagatacagtctcagaagaccaaagggctattgagacttttcaacaaagggtaatatcgggaaacctcctcggattccattgcccagctatctgtcacttcatcaaaaggacagtagaaaaggaaggtggcacctacaaatgccatcattgcgataaaggaaaggctatcgttcaagatgcctctgccgacagtggtcccaaagatggacccccacccacgaggagcatcgtggaaaaagaagacgttccaaccacgtcttcaaagcaagtggattgatgtgatatctccactgacgtaagggatgacgcacaatcccactatccttcgcaagacccttcctctatataaggaagttcatttcatttggagaggactccggtatttttacaacaataccacaacaaaacaaacaacaaacaacattacaatttactattctagtcgaaatggctgagaaagaagcaaatacccatgtcgtcctcttccccttgccaggccaagggcacatcggctcaatgttgaaactggcacagcttctttccaccgccggattctacgtcactttcgtccacaccgaacgcaactaccgtcgctacctcctcacctccacgtccttccacgtccccaagttccggttccgcaccatccccgacggttttcccgacgacgattcccgctcgcccctcccttttctcgagctccaagagtcgctggacacgaaatgtcgggggcattatcgggaattgttggtcgctgtcgacgaccaagaagagtggcccccagtcacttgtgtcgtggctgatcaagctcttccactctcactcgaagttcccgacgagttggggattcctgtaatgatactcgcaccacacagtgcgtgcagtatattgacgagttattcgattccggagcttataaggggaggtgaactccctatcccagatggggccaatatggatgaactattacaaggcgtactgggattggaaggtatcgtgaggcgtagggatatgtccatcagaagcgccaagtccatccaagatccatttcttcaattcgaagtgaaaatgagcaaaaacttgcccagaggaagagctctcatcctgaacactacagaatcgatagactctctttctttgcgacacattcggtcgatctgtcccactacctacgcactcgggcccttccacgtccttctcaggaacataaaagacgagtcccactccgcaagcctttccgaagaggacaggtcctgcatcgcctggctggactcgaaaccgaacaagtccgcggtctacgtgagtttcggtagcctcgccgccatggcgagagaagcatttcttgagtttcagcagggattgctcgacagcgggtattacttcttgtgggtgatccggcccgatatggtggaaggggggctggaagagagcgagctgaccgcgagcgaacaacgctactttgtgaagtgggccccacaggaggaggttcttgcgcacccggcggtagggtgtttcttgacgcacagcggttggaactctacgttggagagtatctttgcgggagtgccgatgatatgttggcctttctttgcggaccagctgattaacagtaggtttgcgagcgaggtgtggaaaattgccttggatatgaaggatttgtgcggaaggagccacgtggagaggatggtgaaggaagttatgagtggagagaaaggcgaagagctaaggaattctagctgcgagatggcagatagggtgaagaagagtgcagaggaaggtggctcttcctacgccaacttcaaagagttggttggacatatcaaatctttgagcttaccagcagaaagaggagaaaatggtggtgaaggaatgagtgtacaagcgccgagtaaacttttcctcctcaacgctgaggacggaaaacatgtccttaaaagtgacgaaccgtcggaacaaaggggtccacaatttaatccaaattttcttcggacctgagcttcggccatgctagagtccgcaaaaatcaccagtctctctctacaaatctatctctctctatttttctccagaataatgtgtgagtagttcccagataagggaattagggttcttatagggtttcgctcatgtgttgagcatataagaaacccttagtatgtatttgtatttgtaaaatacttctatcaataaaatttctaattcctaaaaccaaaatccagtgacctcgctgtcaggagagcgcgagtcggtcccattattgaagcatttatcagggttattgtctcatgagcggatacatatttgaatgtatttagaaaaataaacaaataggggttccgcgcacatttccccgaaaagtgccacctgacgtctaagaaaccattattatcatgacattaacctataaaaataggcgtatcacgaggccctttcgtcttcaagaattagcttggcaattcccgatctagtaacatagatgacaccghgcgcgataatttatcctagtttgcgcgctatattttgttttctatcgcgtattaaatgtataattgcgggactctaatcataaaaacccatctcataaataacgtcatgcattacatgttaattattacatgcttaacgtaattcaacagaaattatatgataatcgtcgcaagaccggcaacaggattcaatcttaagaaactttattgccaaatgtttgaacgatcgggatcgaagatccattccaagctcattcctttgccctcggacgagtgctggggcgtcggtttccactatcggcgagtacttctacacagccatcggtccagacggccgcgcttctgcgggcgatttgtgtacgcccgacagtcccggctccggatcggacgattgcgtcgcatcgaccctgcgcccaagctgcatcatcgaaattgccgtcaaccaagctctgatagagttggtcaagaccaatgcggagcatatacgcccggagtcgtggcgatcctgcaagctccggatgcctccgctcgaagtagcgcgtctgctgctccatacaagccaaccacggcctccagaagaagatgttggcgacctcgtattgggaatccccgaacattgcctcgctccagtcaatgaccgctgttatgcggccattgtccgtcaggacattgttggagccgaaatccgcgtgcacgaggtgccggacttcggggcagtcctcggcccaaagcatcagctcatcgagagcctgcgcgacggacgcactgacggtgtcgtccatcacagtttgccagtgatacacatggggatcagcaatcgcgcatatgaaatcacgccatgtagtgtattgaccgattccttgcggtccgaatgggccgaacccgctcgtctggctaagatcggccgcagcgatcgcatccatggcctccgcgaccggctgcagaacagcgggcagttcggtttcaggcaggtcttgcaacgtgacaccctgtgcacggcgggagatgcaataggtcaggctctcgctgaattccccaatgtcaagcacttccggaatcgggagcgcggccgatgcaaagtgccgataaacataacgatctttgtagaaaccatcggcgcagctatttacccgcaggacatatccacgccctcctacatcgaagctgaaagcacgagattcttcgccctccgagagctgcatcaggtcggacacgctgtcgaacttttcgatcagaaacttctcgacagacgtcgcggtgagttcaggctttttcattgcctcgatcgagttgagagtgaatatgagactctaattggataccgaggggaatttatggaacgtcagtggagcatttttgacaagaaatatttgctagctgatagtgaccttaggcgacttttgaacgcgcaataatggtttctgacgtatgtgcttagctcattaaactccagaaacccgcggctcagtggctccttcaacgttgcggttctgtcagttccaaacgtaaaacggcttgtcccgcgtcatcggcgggggtcataccgtgactcccttaattctcatgtatctccgtcaggaggtcaaacaattttgaggaattcaatttcatctttaactggtacaataatcattttatcatgaaaataagcagctcaagagaatttttgaagaatcttttatttctttaacatttaaccacatgaatttttaatttttttttgcaatacatttaaaccgaaatggtcaaacgatcaaccaactgatctttattctaataaacttctagtttacatttgcatgtgagtgcatcatcattatcatatttgtacacaacaaacaagaaaaaaatataaacaatattttatttaaatatttatattccactttgactgtagatattaaatcttgtcatcatttatagtctcaatattataatttttttattttttcaaaattcaaaagtttacaattatttttttgaactataatattatccaagatgaacatctcaagaagaaaattattaatattgttatggttaaaattttacatacaatacttgttttttgctttacttttatcttaccgtagatacacaatcgacgataacttagtgatcacacaataataattattttgttcatgacacaatatttataagaaatacttatttctttcttttatccttcagtagttcataataaaaacataccataatatttgtgatgcattcatagtacgtaatgaaatgacaatttatgtcaaattattttcttttatactctcaaacctcccgtaaaggtgagatgagtcatttatccaattatacataaatatgtctttattcatgctctttatcacattctgacacattcacttaatttcaagagtaagcaagcatgataactgaaactatttatgcgtatcttaccttgatatttgacacattacatgacacacctcaacatcactttcaaagattaagcgcaccaccatattatctttctttttttttttatgaaggttttataaaattattaaattaggtccaaaaaattgtttgtcaaataaccttttatactagattgatgacaaaaattacctttacgttttgaaagaccattttaagacctaatctatcagtgactccttaaagttggcacaatatttcacttagacaccctaattgaatgatgttcattttaaacacccaatgtagggttccgctatatcattttgacacatttcttaacatcaacaaaaatatataatgagtatgtgatatactcgcgaatgacgtgaaaaatgaagacatttgttatttgtatcaaagtagttactaaataattaattttgaataaaaataaaagctgaccagtaaatcaataacacataatattttccacctaataattaaaatataaaataaaaaagagccatctcagggtcatctgcccaccattgctatttcaaagaaatttgtacgttagtttatagaaattgatgttaaaattctttcaagaaaaatttatgaatgaatttattctctaatttaaaaatattttctgttatttttgttgaaagaaatttaacttggataaaatggtggttaaaactggaaagaagaaaagagaaaaaataattaaaaatcatttcacgctctaatcaatgagcgtatcacattcattatgttatataagcaaaagtgacaaaacgaaaataatatattacatgaaatgtctaaaataaatatcgtctaattaaaatatctaagtaacatattgtgcctaactttagagggatcatcaataagttaaaccccattttaataactcataattgtcctttttatttaatattgtcacaaatcacaatgataattaacattaatttgtcctttgtgacgtccatattcatgcatttaaccaatcatcttcatttggacttattatcacaattatcccactttcctcacaaaatggagcattcaagtggaatagactacacgatttttaatttcatcaaaaacatctttttgctttattcattattatattgtcgctattgttgaattttatttgccctaaatttcttaccataaatagatttttcttttagaaaaaggagattgactaattcttttcttgtaggaaaaggtttaggactctataaatagagacatattccttctaacttaatcaacatttacaatgtagtcttaaagactttgaaagtttttggttagggggagaaattgtgggtcacaagcttgatacgttatcaattgtgtaaacctcccatgtattctgagtgaatttggttgaggttgtttccctctgtattttgtactctcatatttatagtggattgttcatctctttcgtggacgtaggtcgattgaccgtcgattgaccgaaccacgttaaatctttgtattttttgatatatttctcattatcttcttactcgtgatctttcaaggtttgcattgctatcttccgcgttacaccaacttatttacgatcctaacagctatggtgtggaaacataaatcaaacattttactgatataaacacatctttgattataacatgatagaaatttgagcccaactttttatcatcattatatacaaaaagttctaaattttttttttgatgtagtaaaacttaaatccatagtcttgcccctaaaccaatgacataatatataacccaaaatatactagttttcgccctcgagccctttaaaaagtatagtcaatatttacggtgaccgtgaatttcttaattatgatatataatttaaaagaaatcatgatcacattctactgatgagaacatgtgctaatcaagggaaaacatggatgtgaaaaatactttttgttaaaagtaaaaaaaaatgtgaaattttgttagttatttactacctatacattatttgagcatgtgcaaactttacaaatacctaatagaagattttcacctgcctgtatatatgtaaattaattataatgaacactctcacataaaataattatcagtatatacattaatacttgccctccacaatgaattaaataaaatgtagaacatgatctacacttcaataaaactaagaccataaagaataatttcaaaatatacacatgtcaacaataaattatttgcatattatattaacttactaaacaatctttacttttgaaatataaaaataatcaagttataagtctgctcaaagtaaagcacttgttagactcatctgattttgagaaggtaagcaaattgatggtgcataatagtcacaagtaaaatataaaatagatttcattagtaaaattgttttttactttctttatatataattatcaatatccttcaatggtaggttaattatattgttaacttcttgttgaattaaagcaataagacaagaatattaaagataaaagaacaataaaaatagaaagactaagagataagagttttcttattcttctttcaataagtatcatcaagtgtatacaatataaatttttgtatttttgatctatctatttataatgttatatataagcatacaaaagatcagtcataaatatgactttaatcatgaaaataatgaaagagattatgaaggcgtaaggttactagaataatagtcattaaaaaaaggggttatctttataattgaataattgatgaagtaatggagataattagtgagcataaatttttttaaaaaaatggacatttacactataatattttataacactttcccttaaacatctaggtataaataatgagtcttgtcaaaatcttagtaggaaaaattctgtgaaatttttttagtgaaaacaaatgatataaatatcttgaatactcattatttgttgtctcattaaaaatcttatctgacctataaaataaattatttgctcaactcaaaatagtttttcattctaaaattagtataattattagtgaatatttaattaacataattgtatactaaggggcctataaattggattcttctcaaagaaaaataaaatcaccacacaactttcttcttctgctcatcaattagcaattaatccaaaaccaaatggaatctcctgctactaaattacctgcacctctgctgatgttatcttcttctccattccttctcccttctcctaataagagctcctccatcttccttccacgtaaattagggccgctacctccaaaatattattattacaattgctgccatcctaagagtagatcaatctcagtagtatcaatggcaaataaggaggaggcagagacaagtaagaagaagcccaaaccattaaaagtactaattaccaaagtggatccgaagccgaggaagggcatggcatccgtcgcagtggacttactcgagaaggcctttgtatacctattgtccggaaattctgcagctgatcgtagtagtagtagtggtcgtcgtcgtcgtaaagagcattactacctctccggcaattatgcgcccgtcggacacgaaaccccgccctccgaccacctccccattcatggatcccttcctgaatgcttgaatggagtgtttctgagagttggtcctaaccccaagtttgctcccgtagccggatacaattgggtcgatggagatggaatgattcatggattgcgtattaaagatggaaaagcaacttatctatctcgatatattaaaacgtcacggtttaaacaagaagaatattttggaagagcaaaatttatgaagattggagatctaaggggattgcttgggttctttacgatcttaatactagtacttcgaacaacattgaaagtaatagacatttcatatggaagagggacgggtaatacagctcttgtgtatcataatggcttactattggctctatcagaagaagataaaccttatgttgttaaagttttagaagatggagacttgcaaactcttgggatattggattatgacaagaaattgtcacatccattcaccgctcatccaaagatcgatccgttaactgatgagatgtttacctttggatattccatctcgcctccgtatcttacttatcgagtcatttccaaggatggagtgatgcaagatccagtgcaaatctcaattacatcccctaccataatgcatgattttgctattactgaaaattatgccatcttcatggacctgcccttgtatttccaaccagaggaaatggtaaaggggaaatttgtctcttcatttcaccctacaaaaagagctcgtatcggtgtgcttccacgatatgcaaaagacgagcatccaattcgatggttcgatcttccaagttgcttcatgactcataatgcaaatgcttgggaagagaatgatgaagttgtgctattcacatgtcgccttgagagtcctgatcttgacatgcttagtggacctgcggaagaagagattgggaattcaaaaagtgagctttacgaaatgaggttcaatttgaaaactggaattacttcacaaaagcaactatctgtacctagtgttgattttcctcggatcaaccaaagttatactggcaggaaacagcaatatgtttattgtactcttggcaacaccaagattaagggcattgtgaagtttgatctgcaaattgaaccagaagccggaaagacaatgcttgaagttggaggaaatgtacaaggcatctttgagttgggacctagaagatatggttcagaggcaatatttgtgccatgccaacctggcatcaaatctgatgaggatgacggttacttgatattctttgtacacgacgaaaacaatgggaaatctgaggtcaatgtcatcgatgcaaagacaatgtctgcagaacctgtggctgttgtggaacttccaagcagggttccatatggattccatgccttgtttctgaatgaggaagaacttcagaagcaccaagcagagacatgagcttcggccatgctagagtccgcaaaaatcaccagtctctctctacaaatctatctctctctatttttctccagaataatgtgtgagtagttcccagataagggaattagggttcttatagggtttcgctcatgtgttgagcatataagaaacccttagtatgtatttgtatttgtaaaatacttctatcaataaaatttctaattcctaaaaccaaaatccagtgacctcgctgtcatgagacgaattctgacaggatatattggcgggtaaacctaagagaaaagagcgtttattagaataatcggatatttaaaagggcgtgaaaaggtttatccgttcgtccatttgtatgtgcatgccaaccacagggttcccctcgggatcaaagtactttgatccaacccctccgctgctatagtgcagtcggcttctgacgttcagtgcagccgtcatctgaaaacgacatgtcgcacaagtcctaagttacgcgacaggctgccgccctgcccttttcctggcgttttcttgtcgcgtgttttagtcgcataaagtagaatacttgcgactagaaccggagacattacgccatgaacaagagcgccgccgctggcctgctgggctatgcccgcgtcagcaccgacgaccaggacttgaccaaccaacgggccgaactgcacgcggccggctgcaccaagctgttttccgagaagatcaccggcaccaggcgcgaccgcccggagctggccaggatgcttgaccacctacgccctggcgacgttgtgacagtgaccaggctagaccgcctggcccgcagcacccgcgacctactggacattgccgagcgcatccaggaggccggcgcgggcctgcgtagcctggcagagccgtgggccgacaccaccacgccggccggccgcatggtgttgaccgtgttcgccggcattgccgagttcgagcgttccctaatcatcgaccgcacccggagcgggcgcgaggccgccaaggcccgaggcgtgaagtttggcccccgccctaccctcaccccggcacagatcgcgcacgcccgcgagctgatcgaccaggaaggccgcaccgtgaaagaggcggctgcactgcttggcgtgcatcgctcgaccctgtaccgcgcacttgagcgcagcgaggaagtgacgcccaccgaggccaggcggcgcggtgccttccgtgaggacgcattgaccgaggccgacgccctggcggccgccgagaatgaacgccaagaggaacaagcatgaaaccgcaccaggacggccaggacgaaccgtttttcattaccgaagagatcgaggcggagatgatcgcggccgggtacgtgttcgagccgcccgcgcacctctcaaccgtgcggctgcatgaaatcctggccggtttgtctgatgccaagctggcggcctggccggccagcttggccgctgaagaaaccgagcgccgccgtctaaaaaggtgatgtgtatttgagtaaaacagcttgcgtcatgcggtcgctgcgtatatgatccgatgagtaaataaacaaatacgcaaggggaacgcatgaaggttatcgctgtacttaaccagaaaggcgggtcaggcaagacgaccatcggaacccatctagcccgcgccctgcaactcgccggggccgatgttctgttagtcgattccgatccccagggcagtgcccgcgattgggcggccgtgcgggaagatcaaccgctaaccgttgtcggcatcgaccgcccgacgattgaccgcgacgtgaaggccatcggccggcgcgacttcgtagtgatcgacggagcgccccaggcggcggacttggctgtgtccgcgatcaaggcagccgacttcgtgctgattccggtgcagccaagcccttacgacatatgggccaccgccgacctggtggagctggttaagcagcgcattgaggtcacggatggaaggctacaagcggcctttgtcgtgtcgcgggcgatcaaaggcacgcgcatcggcggtgaggttgccgaggcgctggccgggtacgagctgcccattcttgagtcccgtatcacgcagcgcgtgagctacccaggcactgccgccgccggcacaaccgttcttgaatcagaacccgagggcgacgctgcccgcgaggtccaggcgctggccgctgaaattaaatcaaaactcatttgagttaatgaggtaaagagaaaatgagcaaaagcacaaacacgctaagtgccggccgtccgagcgcacgcagcagcaaggctgcaacgttggccagcctggcagacacgccagccatgaagcgggtcaactttcagttgccggcggaggatcacaccaagctgaagatgtacgcggtacgccaaggcaagaccattaccgagctgctatctgaatagatcgcgcagctaccagagtaaatgagcaaatgaataaatgagtagatgaattttagcggctaaaggaggcggcatggaaaatcaagaacaaccaggcaccgacgccgtggaatgccccatgtgtggaggaacgggcggttggccaggcgtaagcggctgggttgtctgccggccctgcaatggcactggaacccccaagcccgaggaatcggcgtgacggtcgcaaaccatccggcccggtacaaatcggcgcggcgctgggtgatgacctggtggagaagttgaaggccgcgcaggccgcccagcggcaacgcatcgaggcagaagcacgccccggtgaatcgtggcaagcggccgctgatcgaatccgcaaagaatcccggcaaccgccggcagccggtgcgccgtcgattaggaagccgcccaagggcgacgagcaaccagattttttcgttccgatgctctatgacgtgggcacccgcgatagtcgcagcatcatggacgtggccgttttccgtctgtcgaagcgtgaccgacgagctggcgaggtgatccgctacgagcttccagacgggcacgtagaggtttccgcagggccggccggcatggccagtgtgtgggattacgacctggtactgatggcggtttcccatctaaccgaatccatgaaccgataccgggaagggaagggagacaagcccggccgcgtgttccgtccacacgttgcggacgtactcaagttctgccggcgagccgatggcggaaagcagaaagacgacctggtagaaacctgcattcggttaaacaccacgcacgttgccatgcagcgtacgaagaaggccaagaacggccgcctggtgacggtatccgagggtgaagccttgattagccgctacaagatcgtaaagagcgaaaccgggcggccggagtacatcgagatcgagctagctgattggatgtaccgcgagatcacagaaggcaagaacccggacgtgctgacggttcaccccgattactttttgatcgatcccggcatcggccgttttctctaccgcctggcacgccgcgccgcaggcaaggcagaagccagatggttgttcaagacgatctacgaacgcagtggcagcgccggagagttcaagaagttctgtttcaccgtgcgcaagctgatcgggtcaaatgacctgccggagtacgatttgaaggaggaggcggggcaggctggcccgatcctagtcatgcgctaccgcaacctgatcgagggcgaagcatccgccggttcctaatgtacggagcagatgctagggcaaattgccctagcaggggaaaaaggtcgaaaaggactctttcctgtggatagcacgtacattgggaacccaaagccgtacattgggaaccggaacccgtacattgggaacccaaagccgtacattgggaaccggtcacacatgtaagtgactgatataaaagagaaaaaaggcgatttttccgcctaaaactctttaaaacttattaaaactcttaaaacccgcctggcctgtgcataactgtctggccagcgcacagccgaagagctgcaaaaagcgcctacccttcggtcgctgcgctccctacgccccgccgcttcgcgtcggcctatcgcggccgctggccgctcaaaaatggctggcctacggccaggcaatctaccagggcgcggacaagccgcgccgtcgccactcgaccgccggcgcccacatcaaggcaccctgcctcgcgcgtttcggtgatgacggtgaaaacctctgacacatgcagctcccggtgacggtcacagcttgtctgtaagcggatgccgggagcagacaagcccgtcagggcgcgtcagcgggtgttggcgggtgtcggggcgcagccatgacccagtcacgtagcgatagcggagtgtatactggcttaactatgcggcatcagagcagattgtactgagagtgcaccatatgcggtgtgaaataccgcacagatgcgtaaggagaaaataccgcatcaggcgctcttccgcttcctcgctcactgactcgctgcgctcggtcgttcggctgcggcgagcggtatcagctcactcaaaggcggtaatacggttatccacagaatcaggggataacgcaggaaagaacatgtgagcaaaaggccagcaaaaggccaggaaccgtaaaaaggccgcgttgctggcgtttttccataggctccgcccccctgacgagcatcacaaaaatcgacgctcaagtcagaggtggcgaaacccgacaggactataaagataccaggcgtttccccctggaagctccctcgtgcgctctcctgttccgaccctgccgcttaccggatacctgtccgcctttctcccttcgggaagcgtggcgctttctcatagctcacgctgtaggtatctcagttcggtgtaggtcgttcgctccaagctgggctgtgtgcacgaaccccccgttcagcccgaccgctgcgccttatccggtaactatcgtcttgagtccaacccggtaagacacgacttatcgccactggcagcagccactggtaacaggattagcagagcgaggtatgtaggcggtgctacagagttcttgaagtggtggcctaactacggctacactagaaggacagtatttggtatctgcgctctgctgaagccagttaccttcggaaaaagagttggtagctcttgatccggcaaacaaaccaccgctggtagcggtggtttttttgtttgcaagcagcagattacgcgcagaaaaaaaggatctcaagaagatcctttgatcttttctacggggtctgacgctcagtggaacgaaaactcacgttaagggattttggtcatgcattctaggtgattagaaaaactcatcgagcatcaaatgaaactgcaatttattcatatcaggattatcaataccatatttttgaaaaagccgtttctgtaatgaaggagaaaactcaccgaggcagttccataggatggcaagatcctggtatcggtctgcgattccgactcgtccaacatcaatacaacctattaatttcccctcgtcaaaaataaggttatcaagtgagaaatcaccatgagtgacgactgaatccggtgagaatggcaaaagtttatgcatttctttccagacttgttcaacaggccagccattacgctcgtcatcaaaatcactcgcatcaaccaaaccgttattcattcgtgattgcgcctgagcgagtcgaaatacgcgatcgctgttaaaaggacaattacaaacaggaatcgaatgcaaccggcgcaggaacactgccagcgcatcaacaatattttcacctgaatcaggatattcttctaatacctggaatgctgttttccctgggatcgcagtggtgagtaaccatgcatcatcaggagtacggataaaatgcttgatggtcggaagaggcataaattccgtcagccagtttagtctgaccatctcatctgtaacatcattggcaacgctacctttgccatgtttcagaaacaactctggcgcatcgggcttcccatacaatcggtagattgtcgcacctgattgcccgacattatcgcgagcccatttatacccatataaatcagcatccatgttggaatttaatcgcggccttgagcaagacgtttcccgttgaatatggctcataacagaacttattatttccttcctcttttctacagtatttaaagataccccaagaagctaattataacaagacgaactccaattcactgttccttgcattctaaaaccttaaataccagaaaacagctttttcaaagttgttttcaaagttggcgtataacatagtatcgacggagccgattttgaaaccgcggtgatcacaggcagcaacgctctgtcatcgttacaatcaacatgctaccctccgcgagatcatccgtgtttcaaacccggcagcttagttgccgttcttccgaatagcatcggtaacatgagcaaagtctgccgccttacaacggctctcccgctgacgccgtcccggactgatgggctgcctgtatcgagtggtgattttgtgccgagctgccggtcggggagctgttggctggctggtggcaggatatattgtggtgtaaacataacgaattcgtctca

SEQ ID NO: 25 - DNA, 21 bp, Artificial Sequence
  CsUGT2 forward primer
tcgagcctagtgatctgccgt

SEQ ID NO: 26 - DNA, 21 bp, Artificial Sequence
  CsUGT2 reverse primer
tcgagccagtccaagtaggga

SEQ ID NO: 27 - DNA, 22 bp, Artificial Sequence
  UGT709G1 forward primer
actcacctccacgtccttccag

SEQ ID NO: 28 - DNA, 21 bp, Artificial Sequence
  UGT709G1 reverse primer
cttgatcagccacgacacaag

SEQ ID NO: 29 - DNA, 20 bp, Artificial Sequence
  CsCCD2L forward primer
acatgtcgccttgagagtcc

SEQ ID NO: 30 - DNA, 20 bp, Artificial Sequence
  CsCCD2L reverse primer
tcagatttgatgccaggttg

SEQ ID NO: 31 - DNA, 21 bp, Artificial Sequence
  Actin-2 forward primer
cattgtgctcagtggtggttc

SEQ ID NO: 32 - DNA, 21 bp, Artificial Sequence
  Actin-2 reverse primer
tctgctggaaggtgctaagtg